European Patent Application EP 4 202 048 A1, published June 28, 2023. Title: Alpharetroviral particles for delivery of RNA into cells. Applicant: Medizinische Hochschule Hannover. The sequence listing filed with the application follows.

SEQUENCE LISTING (62 sequences)

SEQ ID NO: 1 - DNA, 8478 bp, Artificial Sequence
  expression cassette for CMV.ASLV.gag.co.NC.pr.MS2.pA
  promoter 232..819: /note="CMV early promoter"
  gene 232..4302: /gene="expression cassette for aGag-MS2"
  intron 907..1450: /note="beta-globin intron"
  CDS 1462..1914: /note="matrix (MA)" /transl_table=1
  gene 1462..3208: /note="codon-optimized alpharetroviral Gag"
  CDS 1915..1935: /function="protease site" /transl_table=1
  CDS 1936..1986: /note="p2" /transl_table=1
  CDS 1987..2007: /function="protease site" /transl_table=1
  CDS 2008..2172: /note="p10" /transl_table=1
  CDS 2173..2193: /function="protease site" /transl_table=1
  CDS 2194..2919: /note="capsid (CA)" /transl_table=1
  CDS 2920..2940: /function="protease site" /transl_table=1
  CDS 2941..3186: /note="nucleocapsid (NC)" /transl_table=1
  CDS 3187..3207: /function="first linker, protease site" /transl_table=1
  CDS 3208..3222: /function="glycin linker" /transl_table=1
  CDS 3208..3612: /note="MS2 coat protein" /transl_table=1
  CDS 3223..3999: /note="MS2 coat protein dimer (MS2)" /transl_table=1
  misc_feature 3613..3615: /note="Ala as a linker"
  CDS 3616..3999: /note="MS2 coat protein" /transl_table=1
  polyA_signal 4078..4302: /note="bgH poly A signal"
  misc_feature 4348..4776: /note="F1 ori"
  promoter 4790..5119: /note="SV40 promoter"
  CDS 5186..5980: /gene="kanamycin/neomycin resistance gene" /transl_table=1
  polyA_signal 6154..6275: /note="SV40 poly A signal"
  gene 7482..8342: /note="ampicillin resistance gene in antisense orientation"
  promoter 8384..8412: /note="ampicillin resistance gene promoter in antisense orientation"
gacggatcgggagatctcccgatcccctatggtgcactctcagtacaatctgctctgatgccgcatagttaagccagtatctgctccctgcttgtgtgttggaggtcgctgagtagtgcgcgagcaaaatttaagctacaacaaggcaaggcttgaccgacaattgcatgaagaatctgcttagggttaggcgttttgcgctgcttcgcgatgtacgggccagatatacgcgttgacattgattattgactagttattaatagtaatcaattacggggtcattagttcatagcccatatatggagttccgcgttacataacttacggtaaatggcccgcctggctgaccgcccaacgacccccgcccattgacgtcaataatgacgtatgttcccatagtaacgccaatagggactttccattgacgtcaatgggtggactatttacggtaaactgcccacttggcagtacatcaagtgtatcatatgccaagtacgccccctattgacgtcaatgacggtaaatggcccgcctggcattatgcccagtacatgaccttatgggactttcctacttggcagtacatctacgtattagtcatcgctattaccatggtgatgcggttttggcagtacatcaatgggcgtggatagcggtttgactcacggggatttccaagtctccaccccattgacgtcaatgggagtttgttttggcaccaaaatcaacgggactttccaaaatgtcgtaacaactccgccccattgacgcaaatgggcggtaggcgtgtacggtgggaggtctatataagcagagctctctggctaactagagaacccactgcttactggcttatcgaaattaatacgactcactatagggagacccaagcttggtaccgagctcggatcctgagaacttcagggtgagtctatgggacccttgatgttttctttccccttcttttctatggttaagttcatgtcataggaaggggagaagtaacagggtacacatattgaccaaatcagggtaattttgcatttgtaattttaaaaaatgctttcttcttttaatatacttttttgtttatcttatttctaatactttccctaatctctttctttcagggcaataatgatacaatgtatcatgcctctttgcaccattctaaagaataacagtgataatttctgggttaaggcaatagcaatatttctgcatataaatatttctgcatataaattgtaactgatgtaagaggtttcatattgctaatagcagctacaatccagctaccattctgcttttattttatggttgggataaggctggattattctgagtccaagctaggcccttttgctaatcatgttcatacctcttatcttcctcccacagctcctgggcaacgtgctggtctgtgtgctggcccatcactttggcaaagaattcgccaccatggaagccgtgatcaaagtgatcagcagcgcctgcaagacctactgcggcaagatcagccccagcaagaaagaaatcggcgctatgctgtctctcctgcaaaaggaaggcctgctgatgagccccagcgacctgtacagccccggcagctgggatcctatcacagccgccctgagccagagggccatggtgctgggcaagagcggcgagctgaaaacctgggggctggtgctgggagccctgaaggccgccagagaagaacaggtgaccagcgagcaggccaagttttggctgggcctgggcggaggaagagtgtctccccctggccccgagtgtatcgagaagcccgccaccgagcggagaatcgacaagggcgaggaagtgggcgagacaaccgtgcagcgggacgccaagatggcccctgaggaagccgccacccctaagaccgtgggcaccagctgctaccactgtggcaccgccgtgggctgtaattgtgccaccgccaccgcctctgcccctcctcctccttacgtgggcagcggcctgtatccttctctggccggcgtgggcgagcagcagggacagggcgacaataccagcagaggcgccgagcagcctagagaggaacctggacacgctggccaggccccaggacctgccctgacagattgggccagagtgcgggaggaactggcctctaccggaccccctgtggtggccatgcccgtggtgatcaagacagagggccctgcctggacccctctggaacccaagctgatcacccggctggccgatacagtgcggaccaagggcctgagaagccccatcaccatggccgaggtggaggccctgatgagcagccccctgctgccccacgacgtgaccaacctgatgagagtgatcctgggccctgctccctacgccctgtggatggatgcctggggcgtgcagctgcagacagtgatcgccgctgccaccagagatcccagacaccccgccaatggccagggcagaggcgagcggaccaacctggacagactgaagggcctggccgacggcatggtgggcaatcctcagggacaggccgctctgctgaggcctggcgaactggtggccatcacagccagcgccctgcaggccttcagagaggtggccagactggccgagcctgccggcccttgggccgatatcacccagggccccagcgagagcttcgtggacttcgccaaccggctgatcaaggccgtggagggcagcgatctgcctcctagcgccagagcccccgtgatcatcgactgcttccggcagaagtcccagcccgacatccagcagctgatcagagccgcccctagcaccctgaccacccctggcgagatcatcaaatacgtgctggaccggcagaagatcgcccctctgaccgatcagggcattgccgccgctatgagcagcgccatccagcctctggtgatggccgtggtgaacagagagagggacggccagacaggatctggcggcagagccagaggcctgtgctacacctgtggcagccctggccactaccaggcccagtgccccaagaagcggaagtccggcaacagccgggagagatgccagctgtgtgacggcatgggccacaacgccaagcagtgccggaagcgggatggcaatcagggccagaggcccggcagaggactgtctagcggcccttggcctggacctgagcagcctgccgtgagcctggccatgaccggtggcggcggcatggcctccaacttcacccagttcgtgctggtggacaacggcggcacaggcgacgtgacagtggctcccagcaacttcgctaacggcgtggccgagtggatcagcagcaacagcagatcccaggcctacaaagtgacctgcagcgtgcggcagagcagcgcccagaaccggaagtacaccatcaaggtggaagtgcccaaggtggcaacccagacagtgggcggagtggaactgcctgtggccgcttggagaagctacctgaacatggaactgaccatccccatcttcgccaccaacagcgactgcgagctgatcgtgaaggccatgcagggcctgctgaaggacggcaaccctatcccttctgccattgccgccaacagcggcatctacgccaatttcacacagtttgtgctggtcgacaatggcggaactggcgacgtgactgtcgccccaagcaacttcgctaacggggtcgctgaatggatcagctctaactcgcgttcacaggcttacaaagtaacctgtagcgttcgtcagagctctgcgcagaatcgcaaatacaccatcaaagtcgaggtgcctaaagtggcaacccagactgttggtggtgtagagcttcctgtagccgcatggcgttcgtacttaaatatggaactaaccattccaattttcgccacgaattccgactgcgagcttattgttaaggcaatgcaaggtctcctaaaagatggaaacccgattccctcggccatcgcggcaaactccggcatctactgagcggccgctcgagcatgcatctagagggccctattctatagtgtcacctaaatgctagagctcgctgatcagcctcgactgtgccttctagttgccagccatctgttgtttgcccctcccccgtgccttccttgaccctggaaggtgccactcccactgtcctttcctaataaaatgaggaaattgcatcgcattgtctgagtaggtgtcattctattctggggggtggggtggggcaggacagcaagggggaggattgggaagacaatagcaggcatgctggggatgcggtgggctctatggcttctgaggcggaaagaaccagctggggctctagggggtatccccacgcgccctgtagcggcgcattaagcgcggcgggtgtggtggttacgcgcagcgtgaccgctacacttgccagcgccctagcgcccgctcctttcgctttcttcccttcctttctcgccacgttcgccggctttccccgtcaagctctaaatcgggggctccctttagggttccgatttagtgctttacggcacctcgaccccaaaaaacttgattagggtgatggttcacgtagtgggccatcgccctgatagacggtttttcgccctttgacgttggagtccacgttctttaatagtggactcttgttccaaactggaacaacactcaaccctatctcggtctattcttttgatttataagggattttgccgatttcggcctattggttaaaaaatgagctgatttaacaaaaatttaacgcgaattaattctgtggaatgtgtgtcagttagggtgtggaaagtccccaggctccccagcaggcagaagtatgcaaagcatgcatctcaattagtcagcaaccaggtgtggaaagtccccaggctccccagcaggcagaagtatgcaaagcatgcatctcaattagtcagcaaccatagtcccgcccctaactccgcccatcccgcccctaactccgcccagttccgcccattctccgccccatggctgactaattttttttatttatgcagaggccgaggccgcctctgcctctgagctattccagaagtagtgaggaggcttttttggaggcctaggcttttgcaaaaagctcccgggagcttgtatatccattttcggatctgatcaagagacaggatgaggatcgtttcgcatgattgaacaagatggattgcacgcaggttctccggccgcttgggtggagaggctattcggctatgactgggcacaacagacaatcggctgctctgatgccgccgtgttccggctgtcagcgcaggggcgcccggttctttttgtcaagaccgacctgtccggtgccctgaatgaactgcaggacgaggcagcgcggctatcgtggctggccacgacgggcgttccttgcgcagctgtgctcgacgttgtcactgaagcgggaagggactggctgctattgggcgaagtgccggggcaggatctcctgtcatctcaccttgctcctgccgagaaagtatccatcatggctgatgcaatgcggcggctgcatacgcttgatccggctacctgcccattcgaccaccaagcgaaacatcgcatcgagcgagcacgtactcggatggaagccggtcttgtcgatcaggatgatctggacgaagagcatcaggggctcgcgccagccgaactgttcgccaggctcaaggcgcgcatgcccgacggcgaggatctcgtcgtgacccatggcgatgcctgcttgccgaatatcatggtggaaaatggccgcttttctggattcatcgactgtggccggctgggtgtggcggaccgctatcaggacatagcgttggctacccgtgatattgctgaagagcttggcggcgaatgggctgaccgcttcctcgtgctttacggtatcgccgctcccgattcgcagcgcatcgccttctatcgccttcttgacgagttcttctgagcgggactctggggttcgaaatgaccgaccaagcgacgcccaacctgccatcacgagatttcgattccaccgccgccttctatgaaaggttgggcttcggaatcgttttccgggacgccggctggatgatcctccagcgcggggatctcatgctggagttcttcgcccaccccaacttgtttattgcagcttataatggttacaaataaagcaatagcatcacaaatttcacaaataaagcatttttttcactgcattctagttgtggtttgtccaaactcatcaatgtatcttatcatgtctgtataccgtcgacctctagctagagcttggcgtaatcatggtcatagctgtttcctgtgtgaaattgttatccgctcacaattccacacaacatacgagccggaagcataaagtgtaaagcctggggtgcctaatgagtgagctaactcacattaattgcgttgcgctcactgcccgctttccagtcgggaaacctgtcgtgccagctgcattaatgaatcggccaacgcgcggggagaggcggtttgcgtattgggcgctcttccgcttcctcgctcactgactcgctgcgctcggtcgttcggctgcggcgagcggtatcagctcactcaaaggcggtaatacggttatccacagaatcaggggataacgcaggaaagaacatgtgagcaaaaggccagcaaaaggccaggaaccgtaaaaaggccgcgttgctggcgtttttccataggctccgcccccctgacgagcatcacaaaaatcgacgctcaagtcagaggtggcgaaacccgacaggactataaagataccaggcgtttccccctggaagctccctcgtgcgctctcctgttccgaccctgccgcttaccggatacctgtccgcctttctcccttcgggaagcgtggcgctttctcatagctcacgctgtaggtatctcagttcggtgtaggtcgttcgctccaagctgggctgtgtgcacgaaccccccgttcagcccgaccgctgcgccttatccggtaactatcgtcttgagtccaacccggtaagacacgacttatcgccactggcagcagccactggtaacaggattagcagagcgaggtatgtaggcggtgctacagagttcttgaagtggtggcctaactacggctacactagaagaacagtatttggtatctgcgctctgctgaagccagttaccttcggaaaaagagttggtagctcttgatccggcaaacaaaccaccgctggtagcggtttttttgtttgcaagcagcagattacgcgcagaaaaaaaggatctcaagaagatcctttgatcttttctacggggtctgacgctcagtggaacgaaaactcacgttaagggattttggtcatgagattatcaaaaaggatcttcacctagatccttttaaattaaaaatgaagttttaaatcaatctaaagtatatatgagtaaacttggtctgacagttaccaatgcttaatcagtgaggcacctatctcagcgatctgtctatttcgttcatccatagttgcctgactccccgtcgtgtagataactacgatacgggagggcttaccatctggccccagtgctgcaatgataccgcgagacccacgctcaccggctccagatttatcagcaataaaccagccagccggaagggccgagcgcagaagtggtcctgcaactttatccgcctccatccagtctattaattgttgccgggaagctagagtaagtagttcgccagttaatagtttgcgcaacgttgttgccattgctacaggcatcgtggtgtcacgctcgtcgtttggtatggcttcattcagctccggttcccaacgatcaaggcgagttacatgatcccccatgttgtgcaaaaaagcggttagctccttcggtcctccgatcgttgtcagaagtaagttggccgcagtgttatcactcatggttatggcagcactgcataattctcttactgtcatgccatccgtaagatgcttttctgtgactggtgagtactcaaccaagtcattctgagaatagtgtatgcggcgaccgagttgctcttgcccggcgtcaatacgggataataccgcgccacatagcagaactttaaaagtgctcatcattggaaaacgttcttcggggcgaaaactctcaaggatcttaccgctgttgagatccagttcgatgtaacccactcgtgcacccaactgatcttcagcatcttttactttcaccagcgtttctgggtgagcaaaaacaggaaggcaaaatgccgcaaaaaagggaataagggcgacacggaaatgttgaatactcatactcttcctttttcaatattattgaagcatttatcagggttattgtctcatgagcggatacatatttgaatgtatttagaaaaataaacaaataggggttccgcgcacatttccccgaaaagtgccacctgacgtc

SEQ ID NO: 2 - DNA, 6338 bp, Artificial Sequence
  expression cassette for GOI.TS Flp recombinase
  promoter 1..589: /note="human CMV immediate early promoter"
  gene 1..3149: /gene="expression cassette for Flp recombinase-TS2-PRE-pA"
  enhancer 59..465: /note="enhancer region"
  TATA_signal 554..560: /note="TATA box"
  misc_feature 583: /note="transcription start point"
  CDS 612..1910: /gene="mouse codon-optimized flp recombinase" /transl_table=1
  protein_bind 1912..2045: /function="MS2 target site (2xTS)"
  protein_bind 1943..1965: /function="target site (TS) hairpin"
  protein_bind 1982..2004: /function="target site (TS) hairpin"
  misc_feature 2046..2974: /note="PRE"
  polyA_signal 3115..3120: /note="SV40 mRNA pA"
  polyA_signal 3144..3149: /note="SV40 mRNA pA"
  misc_feature 3212..3667: /note="FI single-strand DNA origin in antisense orientation"
  promoter 3729..3757: /note="bacterial beta-lactamase promoter for expressing the kanamycin resistance gene"
  promoter 3825..4070: /note="SV40 early promoter, overlaps with SV40 ori at nt 4070"
  misc_feature 4008..4143: /note="SV40 origin of replication"
  gene 4192..4986: /gene="kanamycin/neomycin resistance"
  polyA_signal 5218..5264: /note="herpes simplex virus (HSV) thymidine kinase (TK) poly adenylation signal"
  misc_feature 5571..6214: /note="pUC plasmid replication origin"
tagttattaatagtaatcaattacggggtcattagttcatagcccatatatggagttccgcgttacataacttacggtaaatggcccgcctggctgaccgcccaacgacccccgcccattgacgtcaataatgacgtatgttcccatagtaacgccaatagggactttccattgacgtcaatgggtggagtatttacggtaaactgcccacttggcagtacatcaagtgtatcatatgccaagtacgccccctattgacgtcaatgacggtaaatggcccgcctggcattatgcccagtacatgaccttatgggactttcctacttggcagtacatctacgtattagtcatcgctattaccatggtgatgcggttttggcagtacatcaatgggcgtggatagcggtttgactcacggggatttccaagtctccaccccattgacgtcaatgggagtttgttttggcaccaaaatcaacgggactttccaaaatgtcgtaacaactccgccccattgacgcaaatgggcggtaggcgtgtacggtgggaggtctatataagcagagctggtttagtgaaccgtcagatccgctagcgctaccggtgccaccatggctcctaagaagaagaggaaggtgatgagccagttcgacatcctgtgcaagaccccccccaaggtgctggtgcggcagttcgtggagagattcgagaggcccagcggcgagaagatcgccagctgtgccgccgagctgacctacctgtgctggatgatcacccacaacggcaccgccatcaagagggccaccttcatgagctacaacaccatcatcagcaacagcctgagcttcgacatcgtgaacaagagcctgcagttcaagtacaagacccagaaggccaccatcctggaggccagcctgaagaagctgatccccgcctgggagttcaccatcatcccttacaacggccagaagcaccagagcgacatcaccgacatcgtgtccagcctgcagctgcagttcgagagcagcgaggaggccgacaagggcaacagccacagcaagaagatgctgaaggccctgctgtccgagggcgagagcatctgggagatcaccgagaagatcctgaacagcttcgagtacaccagcaggttcaccaagaccaagaccctgtaccagttcctgttcctggccacattcatcaactgcggcaggttcagcgacatcaagaacgtggaccccaagagcttcaagctggtgcagaacaagtacctgggcgtgatcattcagtgcctggtgaccgagaccaagacaagcgtgtccaggcacatctactttttcagcgccagaggcaggatcgaccccctggtgtacctggacgagttcctgaggaacagcgagcccgtgctgaagagagtgaacaggaccggcaacagcagcagcaacaagcaggagtaccagctgctgaaggacaacctggtgcgcagctacaacaaggccctgaagaagaacgccccctaccccatcttcgctatcaagaacggccctaagagccacatcggcaggcacctgatgaccagctttctgagcatgaagggcctgaccgagctgacaaacgtggtgggcaactggagcgacaagagggcctccgccgtggccaggaccacctacacccaccagatcaccgccatccccgaccactacttcgccctggtgtccaggtactacgcctacgaccccatcagcaaggagatgatcgccctgaaggacgagaccaaccccatcgaggagtggcagcacatcgagcagctgaagggcagcgccgagggcagcatcagataccccgcctggaacggcatcatcagccaggaggtgctggactacctgagcagctacatcaacaggcggatctgagtcgagagatcctaaggtacctaattgcctagaaaacatgaggatcacccatgtctgcaggtcgactctagaaaacatgaggatcacccatgtctgcagtattcccgggttcattagatcctaaggtaccgaattcgagcatcttaccgccatttattcccatatttgttctgtttttcttgatttgggtatacatttaaatgttaataaaacaaaatggtggggcaatcatttacattttatgggatatgtaattactagttcaggtgtattgccacaagacaaacatgttaagaaactttcccgttatttacgctctgttcctgttaatcaacctctggattacaaaatttgtgaaagattgactgatattcttaactatgttgctccttttacgctgtgtggatatgctgctttaatgcctctgtatcatgctattgcttcccgtacggctttcgttttctcctccttgtataaatcctggttgctgtctctttatgaggagttgtggcccgttgtccgtcaacgtggcgtggtgtgctctgtgtttgctgacgcaacccccactggctggggcattgccaccacctgtcaactcctttctgggactttcgctttccccctcccgatcgccacggcagaactcatcgccgcctgccttgcccgctgctggacaggggctaggttgctgggcactgataattccgtggtgttgtcggggaagctgacgtcctttccatggctgctcgcctgtgttgccaactggatcctgcgcgggacgtccttctgctacgtcccttcggctctcaatccagcggacctcccttcccgaggccttctgccggttctgcggcctctcccgcgtcttcgctttcggcctccgacgagtcggatctccctttgggccgcctccccgcctgtttcgcctcggcgtccggtccgtgttgcttggtcgtcacctgtgcagaattgcgaaccatggattccaccgtgaactttgtctcctggcatgcaaatcgtcaacttggcatgccaagaattcggatccaagcttcgaattctgcagtcgacggtaccgcgggcccgggatccaccggatctagataactgatcataatcagccataccacatttgtagaggttttacttgctttaaaaaacctcccacacctccccctgaacctgaaacataaaatgaatgcaattgttgttgttaacttgtttattgcagcttataatggttacaaataaagcaatagcatcacaaatttcacaaataaagcatttttttcactgcattctagttgtggtttgtccaaactcatcaatgtatcttaacgcgtaaattgtaagcgttaatattttgttaaaattcgcgttaaatttttgttaaatcagctcattttttaaccaataggccgaaatcggcaaaatcccttataaatcaaaagaatagaccgagatagggttgagtgttgttccagtttggaacaagagtccactattaaagaacgtggactccaacgtcaaagggcgaaaaaccgtctatcagggcgatggcccactacgtgaaccatcaccctaatcaagttttttggggtcgaggtgccgtaaagcactaaatcggaaccctaaagggagcccccgatttagagcttgacggggaaagccggcgaacgtggcgagaaaggaagggaagaaagcgaaaggagcgggcgctagggcgctggcaagtgtagcggtcacgctgcgcgtaaccaccacacccgccgcgcttaatgcgccgctacagggcgcgtcaggtggcacttttcggggaaatgtgcgcggaacccctatttgtttatttttctaaatacattcaaatatgtatccgctcatgagacaataaccctgataaatgcttcaataatattgaaaaaggaagagtcctgaggcggaaagaaccagctgtggaatgtgtgtcagttagggtgtggaaagtccccaggctccccagcaggcagaagtatgcaaagcatgcatctcaattagtcagcaaccaggtgtggaaagtccccaggctccccagcaggcagaagtatgcaaagcatgcatctcaattagtcagcaaccatagtcccgcccctaactccgcccatcccgcccctaactccgcccagttccgcccattctccgccccatggctgactaattttttttatttatgcagaggccgaggccgcctcggcctctgagctattccagaagtagtgaggaggcttttttggaggcctaggcttttgcaaagatcgatcaagagacaggatgaggatcgtttcgcatgattgaacaagatggattgcacgcaggttctccggccgcttgggtggagaggctattcggctatgactgggcacaacagacaatcggctgctctgatgccgccgtgttccggctgtcagcgcaggggcgcccggttctttttgtcaagaccgacctgtccggtgccctgaatgaactgcaagacgaggcagcgcggctatcgtggctggccacgacgggcgttccttgcgcagctgtgctcgacgttgtcactgaagcgggaagggactggctgctattgggcgaagtgccggggcaggatctcctgtcatctcaccttgctcctgccgagaaagtatccatcatggctgatgcaatgcggcggctgcatacgcttgatccggctacctgcccattcgaccaccaagcgaaacatcgcatcgagcgagcacgtactcggatggaagccggtcttgtcgatcaggatgatctggacgaagagcatcaggggctcgcgccagccgaactgttcgccaggctcaaggcgagcatgcccgacggcgaggatctcgtcgtgacccatggcgatgcctgcttgccgaatatcatggtggaaaatggccgcttttctggattcatcgactgtggccggctgggtgtggcggaccgctatcaggacatagcgttggctacccgtgatattgctgaagagcttggcggcgaatgggctgaccgcttcctcgtgctttacggtatcgccgctcccgattcgcagcgcatcgccttctatcgccttcttgacgagttcttctgagcgggactctggggttcgaaatgaccgaccaagcgacgcccaacctgccatcacgagatttcgattccaccgccgccttctatgaaaggttgggcttcggaatcgttttccgggacgccggctggatgatcctccagcgcggggatctcatgctggagttcttcgcccaccctagggggaggctaactgaaacacggaaggagacaataccggaaggaacccgcgctatgacggcaataaaaagacagaataaaacgcacggtgttgggtcgtttgttcataaacgcggggttcggtcccagggctggcactctgtcgataccccaccgagaccccattggggccaatacgcccgcgtttcttccttttccccaccccaccccccaagttcgggtgaaggcccagggctcgcagccaacgtcggggcggcaggccctgccatagcctcaggttactcatatatactttagattgatttaaaacttcatttttaatttaaaaggatctaggtgaagatcctttttgataatctcatgaccaaaatcccttaacgtgagttttcgttccactgagcgtcagaccccgtagaaaagatcaaaggatcttcttgagatcctttttttctgcgcgtaatctgctgcttgcaaacaaaaaaaccaccgctaccagcggtggtttgtttgccggatcaagagctaccaactctttttccgaaggtaactggcttcagcagagcgcagataccaaatactgtccttctagtgtagccgtagttaggccaccacttcaagaactctgtagcaccgcctacatacctcgctctgctaatcctgttaccagtggctgctgccagtggcgataagtcgtgtcttaccgggttggactcaagacgatagttaccggataaggcgcagcggtcgggctgaacggggggttcgtgcacacagcccagcttggagcgaacgacctacaccgaactgagatacctacagcgtgagctatgagaaagcgccacgcttcccgaagggagaaaggcggacaggtatccggtaagcggcagggtcggaacaggagagcgcacgagggagcttccagggggaaacgcctggtatctttatagtcctgtcgggtttcgccacctctgacttgagcgtcgatttttgtgatgctcgtcaggggggcggagcctatggaaaaacgccagcaacgcggcctttttacggttcctggccttttgctggccttttgctcacatgttctttcctgcgttatcccctgattctgtggataaccgtattaccgccatgcat

SEQ ID NO: 3 - DNA, 5044 bp, Artificial Sequence
  expression cassette for DsRedexp with sgRNA and 2xTS
  promoter 1..589
  enhancer 59..465: /note="enhancer region"
  TATA_signal 554..650: /note="TATA box"
  misc_feature 583: /note="transcription start point"
  CDS 628..1305: /note="human codon-optimized DsRed-Express protein" /transl_table=1
  promoter 1313..1556: /note="human U6 promoter"
  TATA_signal 1533..1665: /note="TATA box"
  misc_feature 1560..1668: /note="BsmBI stuffer"
  misc_feature 1665..1800: /note="sgRNA integrated with 2x TS "
  protein_bind 1681..1701: /function="target site (TS) hairpin"
  protein_bind 1751..1771: /function="target site (TS) hairpin"
  terminator 1801..1806: /note="termination signal"
  polyA_signal 1863..1868: /note="SV40 early mRNA polyadenylation signal"
  polyA_signal 1892..1897: /note="SV40 early mRNA polyadenylation signal"
  misc_feature 1960..2415: /note="F1 single-strand DNA origin in antisense orientation"
  promoter 2477..2505: /note="bacterial beta-lactamase promoter for expressing the kanamycin resistance gene"
  promoter 2573..2818: /note="SV40 early promoter,overlaps with SV40 ori at nt 2818"
  misc_feature 2756..2891: /note="SV40 origin of replication"
  gene 2940..3734: /gene="kanamycin/neomycin resistance"
  polyA_signal 3966..4012: /note="herpes simplex virus (HSV) thymidine kinase (TK) poly adenylation signal"
  misc_feature 4319..4962: /note="pUC plasmid replication origin"
tagttattaatagtaatcaattacggggtcattagttcatagcccatatatggagttccgcgttacataacttacggtaaatggcccgcctggctgaccgcccaacgacccccgcccattgacgtcaataatgacgtatgttcccatagtaacgccaatagggactttccattgacgtcaatgggtggagtatttacggtaaactgcccacttggcagtacatcaagtgtatcatatgccaagtacgccccctattgacgtcaatgacggtaaatggcccgcctggcattatgcccagtacatgaccttatgggactttcctacttggcagtacatctacgtattagtcatcgctattaccatggtgatgcggttttggcagtacatcaatgggcgtggatagcggtttgactcacggggatttccaagtctccaccccattgacgtcaatgggagtttgttttggcaccaaaatcaacgggactttccaaaatgtcgtaacaactccgccccattgacgcaaatgggcggtaggcgtgtacggtgggaggtctatataagcagagctggtttagtgaaccgtcagatccgctagcgctaccggactcagatccaccggtcgccaccatggcctcctccgaggacgtcatcaaggagttcatgcgcttcaaggtgcgcatggagggctccgtgaacggccacgagttcgagatcgagggcgagggcgagggccgcccctacgagggcacccagaccgccaagctgaaggtgaccaagggcggccccctgcccttcgcctgggacatcctgtccccccagttccagtacggctccaaggtgtacgtgaagcaccccgccgacatccccgactacaagaagctgtccttccccgagggcttcaagtgggagcgcgtgatgaacttcgaggacggcggcgtggtgaccgtgacccaggactcctccctgcaggacggctccttcatctacaaggtgaagttcatcggcgtgaacttcccctccgacggccccgtaatgcagaagaagactatgggctgggaggcctccaccgagcgcctgtacccccgcgacggcgtgctgaagggcgagatccacaaggccctgaagctgaaggacggcggccactacctggtggagttcaagtccatctacatggccaagaagcccgtgcagctgcccggctactactacgtggactccaagctggacatcacctcccacaacgaggactacaccatcgtggagcagtacgagcgcgccgagggccgccaccacctgttcctgtagcggccgcgagagggcctatttcccatgattccttcatatttgcatatacgatacaaggctgttagagagataattagaattaatttgactgtaaacacaaagatattagtacaaaatacgtgacgtagaaagtaataatttcttgggtagtttgcagttttaaaattatgttttaaaatggactatcatatgcttaccgtaacttgaaagtatttcgatttcttggctttatatatcttgtggaaaggacgaaacaccggagacggttgtaaatgagcacacaaaatacacatgctaaaatattatattctatgatttttaaatcttttttagcttcttgctcttttttgtacgtctctgttttagagctaggccaacatgaggatcacccatgtctgcagggcctagcaagttaaaataaggctagtccgttatcaacttggccaacatgaggatcacccatgtctgcagggccaagtggcaccgagtcggtgcttttttgaattctaccggaattgttgttgttaacttgtttattgcagcttataatggttacaaataaagcaatagcatcacaaatttcacaaataaagcatttttttcactgcattctagttgtggtttgtccaaactcatcaatgtatcttaaggcgtaaattgtaagcgttaatattttgttaaaattcgcgttaaatttttgttaaatcagctcattttttaaccaataggccgaaatcggcaaaatcccttataaatcaaaagaatagaccgagatagggttgagtgttgttccagtttggaacaagagtccactattaaagaacgtggactccaacgtcaaagggcgaaaaaccgtctatcagggcgatggcccactacgtgaaccatcaccctaatcaagttttttggggtcgaggtgccgtaaagcactaaatcggaaccctaaagggagcccccgatttagagcttgacggggaaagccggcgaacgtggcgagaaaggaagggaagaaagcgaaaggagcgggcgctagggcgctggcaagtgtagcggtcacgctgcgcgtaaccaccacacccgccgcgcttaatgcgccgctacagggcgcgtcaggtggcacttttcggggaaatgtgcgcggaacccctatttgtttatttttctaaatacattcaaatatgtatccgctcatgagacaataaccctgataaatgcttcaataatattgaaaaaggaagagtcctgaggcggaaagaaccagctgtggaatgtgtgtcagttagggtgtggaaagtccccaggctccccagcaggcagaagtatgcaaagcatgcatctcaattagtcagcaaccaggtgtggaaagtccccaggctccccagcaggcagaagtatgcaaagcatgcatctcaattagtcagcaaccatagtcccgcccctaactccgcccatcccgcccctaactccgcccagttccgcccattctccgccccatggctgactaattttttttatttatgcagaggccgaggccgcctcggcctctgagctattccagaagtagtgaggaggcttttttggaggcctaggcttttgcaaagatcgatcaagagacaggatgaggatcgtttcgcatgattgaacaagatggattgcacgcaggttctccggccgcttgggtggagaggctattcggctatgactgggcacaacagacaatcggctgctctgatgccgccgtgttccggctgtcagcgcaggggcgcccggttctttttgtcaagaccgacctgtccggtgccctgaatgaactgcaagacgaggcagcgcggctatcgtggctggccacgacgggcgttccttgcgcagctgtgctcgacgttgtcactgaagcgggaagggactggctgctattgggcgaagtgccggggcaggatctcctgtcatctcaccttgctcctgccgagaaagtatccatcatggctgatgcaatgcggcggctgcatacgcttgatccggctacctgcccattcgaccaccaagcgaaacatcgcatcgagcgagcacgtactcggatggaagccggtcttgtcgatcaggatgatctggacgaagagcatcaggggctcgcgccagccgaactgttcgccaggctcaaggcgagcatgcccgacggcgaggatctcgtcgtgacccatggcgatgcctgcttgccgaatatcatggtggaaaatggccgcttttctggattcatcgactgtggccggctgggtgtggcggaccgctatcaggacatagcgttggctacccgtgatattgctgaagagcttggcggcgaatgggctgaccgcttcctcgtgctttacggtatcgccgctcccgattcgcagcgcatcgccttctatcgccttcttgacgagttcttctgagcgggactctggggttcgaaatgaccgaccaagcgacgcccaacctgccatcacgagatttcgattccaccgccgccttctatgaaaggttgggcttcggaatcgttttccgggacgccggctggatgatcctccagcgcggggatctcatgctggagttcttcgcccaccctagggggaggctaactgaaacacggaaggagacaataccggaaggaacccgcgctatgacggcaataaaaagacagaataaaacgcacggtgttgggtcgtttgttcataaacgcggggttcggtcccagggctggcactctgtcgataccccaccgagaccccattggggccaatacgcccgcgtttcttccttttccccaccccaccccccaagttcgggtgaaggcccagggctcgcagccaacgtcggggcggcaggccctgccatagcctcaggttactcatatatactttagattgatttaaaacttcatttttaatttaaaaggatctaggtgaagatcctttttgataatctcatgaccaaaatcccttaacgtgagttttcgttccactgagcgtcagaccccgtagaaaagatcaaaggatcttcttgagatcctttttttctgcgcgtaatctgctgcttgcaaacaaaaaaaccaccgctaccagcggtggtttgtttgccggatcaagagctaccaactctttttccgaaggtaactggcttcagcagagcgcagataccaaatactgtccttctagtgtagccgtagttaggccaccacttcaagaactctgtagcaccgcctacatacctcgctctgctaatcctgttaccagtggctgctgccagtggcgataagtcgtgtcttaccgggttggactcaagacgatagttaccggataaggcgcagcggtcgggctgaacggggggttcgtgcacacagcccagcttggagcgaacgacctacaccgaactgagatacctacagcgtgagctatgagaaagcgccacgcttcccgaagggagaaaggcggacaggtatccggtaagcggcagggtcggaacaggagagcgcacgagggagcttccagggggaaacgcctggtatctttatagtcctgtcgggtttcgccacctctgacttgagcgtcgatttttgtgatgctcgtcaggggggcggagcctatggaaaaacgccagcaacgcggcctttttacggttcctggccttttgctggccttttgctcacatgttctttcctgcgttatcccctgattctgtggataaccgtattaccgccatgcat

SEQ ID NO: 4 - DNA, 6066 bp, Artificial Sequence
  expression cassette for VSVg
  promoter 654..5971: /note="human CMV immediate early promoter in antisense orientation"
  intron 685..1233: /note="beta-globin intron"
  CDS 1241..2776: /note="VSVg" /transl_table=1
  polyA_signal 2977..3371: /note="beta-globin poly adenylation signal"
  promoter 3824..3852: /note="ampicillin resistance gene promoter element"
  gene 3894..4754: /gene="ampicillin resistance gene"
  misc_feature 5171..5402: /note="pMB1 ori"
actagttattaatagtaatcaattacggggtcattagttcatagcccatatatggagttccgcgttacataacttacggtaaatggcccgcctggctgaccgcccaacgacccccgcccattgacgtcaataatgacgtatgttcccatagtaacgccaatagggactttccattgacgtcaatgggtggagtatttacggtaaactgcccacttggcagtacatcaagtgtatcatatgccaagtacgccccctattgacgtcaatgacggtaaatggcccgcctggcattatgcccagtacatgaccttatgggactttcctacttggcagtacatctacgtattagtcatcgctattaccatggtgatgcggttttggcagtacatcaatgggcgtggatagcggtttgactcacggggatttccaagtctccaccccattgacgtcaatgggagtttgttttggcaccaaaatcaacgggactttccaaaatgtcgtaacaactccgccccattgacgcaaatgggcggtaggcgtgtacggtgggaggtctatataagcagagctcgtttagtgaaccgtcagatcgcctggagacgccatccacgctgttttgacctccatagaagacaccgggaccgatccagcctcccctcgaagcttacatgtggtaccgagctcggatcctgagaacttcagggtgagtctatgggacccttgatgttttctttccccttcttttctatggttaagttcatgtcataggaaggggagaagtaacagggtacacatattgaccaaatcagggtaattttgcatttgtaattttaaaaaatgctttcttcttttaatatacttttttgtttatcttatttctaatactttccctaatctctttctttcagggcaataatgatacaatgtatcatgcctctttgcaccattctaaagaataacagtgataatttctgggttaaggcaatagcaatatttctgcatataaatatttctgcatataaattgtaactgatgtaagaggtttcatattgctaatagcagctacaatccagctaccattctgcttttattttatggttgggataaggctggattattctgagtccaagctaggcccttttgctaatcatgttcatacctcttatcttcctcccacagctcctgggcaacgtgctggtctgtgtgctggcccatcactttggcaaagaattctgacactatgaagtgccttttgtacttagcctttttattcattggggtgaattgcaagttcaccatagtttttccacacaaccaaaaaggaaactggaaaaatgttccttctaattaccattattgcccgtcaagctcagatttaaattggcataatgacttaataggcacagccttacaagtcaaaatgcccaagagtcacaaggctattcaagcagacggttggatgtgtcatgcttccaaatgggtcactacttgtgatttccgctggtatggaccgaagtatataacacattccatccgatccttcactccatctgtagaacaatgcaaggaaagcattgaacaaacgaaacaaggaacttggctgaatccaggcttccctcctcaaagttgtggatatgcaactgtgacggatgccgaagcagtgattgtccaggtgactcctcaccatgtgctggttgatgaatacacaggagaatgggttgattcacagttcatcaacggaaaatgcagcaattacatatgccccactgtccataactctacaacctggcattctgactataaggtcaaagggctatgtgattctaacctcatttccatggacatcaccttcttctcagaggacggagagctatcatccctgggaaaggagggcacagggttcagaagtaactactttgcttatgaaactggaggcaaggcctgcaaaatgcaatactgcaagcattggggagtcagactcccatcaggtgtctggttcgagatggctgataaggatctctttgctgcagccagattccctgaatgcccagaagggtcaagtatctctgctccatctcagacctcagtggatgtaagtctaattcaggacgttgagaggatcttggattattccctctgccaagaaacctggagcaaaatcagagcgggtcttccaatctctccagtggatctcagctatcttgctcctaaaaacccaggaaccggtcctgctttcaccataatcaatggtaccctaaaatactttgagaccagatacatcagagtcgatattgctgctccaatcctctcaagaatggtcggaatgatcagtggaactaccacagaaagggaactgtgggatgactgggcaccatatgaagacgtggaaattggacccaatggagttctgaggaccagttcaggatataagtttcctttatacatgattggacatggtatgttggactccgatcttcatcttagctcaaaggctcaggtgttcgaacatcctcacattcaagacgctgcttcgcaacttcctgatgatgagagtttattttttggtgatactgggctatccaaaaatccaatcgagcttgtagaaggttggttcagtagttggaaaagctctattgcctcttttttctttatcatagggttaatcattggactattcttggttctccgagttggtatccatctttgcattaaattaaagcacaccaagaaaagacagatttatacagacatagagatgaaccgacttggaaagtaactcaaatcctgcacaacagattcttcatgtttggaccaaatcaacttgtgataccatgctcaaagaggcctcaattatatttgagtttttaatttttatgaaaaaaaaaaaaaaaaacggaattcaccccaccagtgcaggctgcctatcagaaagtggtggctggtgtggctaatgccctggcccacaagtatcactaagctcgctttcttgctgtccaatttctattaaaggttcctttgttccctaagtccaactactaaactgggggatattatgaagggccttgagcatctggattctgcctaataaaaaacatttattttcattgcaatgatgtatttaaattatttctgaatattttactaaaaagggaatgtgggaggtcagtgcatttaaaacataaagaaatgaagagctagttcaaaccttgggaaaatacactatatcttaaactccatgaaagaaggtgaggctgcaaacagctaatgcacattggcaacagcccctgatgcctatgccttattcatccctcagaaaaggattcaagtagaggcttgatttggaggttaaagttttgctatgctgtattttacattacttattgttttagctgtcctcatgaatgtcttttcactacccatttgcttatcctgcatctctcagccttgactccactcagttctcttgcttagagataccacctttcccctgaagtgttccttccatgttttacggcgagatggtttctcctcgcctggccactcagccttagttgtctctgttgtcttatagaggtctacttgaagaaggaaaaacagggggcatggtttgactgtcctgtgagcccttcttccctgcctcccccactcacagtgacccggaatccctcgacatggcagtctagaattcttgaagacgaaagggcctcgtgatacgcctatttttataggttaatgtcatgataataatggtttcttagacgtcaggtggcacttttcggggaaatgtgcgcggaacccctatttgtttatttttctaaatacattcaaatatgtatccgctcatgagacaataaccctgataaatgcttcaataatattgaaaaaggaagagtatgagtattcaacatttccgtgtcgcccttattcccttttttgcggcattttgccttcctgtttttgctcacccagaaacgctggtgaaagtaaaagatgctgaagatcagttgggtgcacgagtgggttacatcgaactggatctcaacagcggtaagatccttgagagttttcgccccgaagaacgttttccaatgatgagcacttttaaagttctgctatgtggcgcggtattatcccgtgttgacgccgggcaagagcaactcggtcgccgcatacactattctcagaatgacttggttgagtactcaccagtcacagaaaagcatcttacggatggcatgacagtaagagaattatgcagtgctgccataaccatgagtgataacactgcggccaacttacttctgacaacgatcggaggaccgaaggagctaaccgcttttttgcacaacatgggggatcatgtaactcgccttgatcgttgggaaccggagctgaatgaagccataccaaacgacgagcgtgacaccacgatgcctgcagcaatggcaacaacgttgcgcaaactattaactggcgaactacttactctagcttcccggcaacaattaatagactggatggaggcggataaagttgcaggaccacttctgcgctcggcccttccggctggctggtttattgctgataaatctggagccggtgagcgtgggtctcgcggtatcattgcagcactggggccagatggtaagccctcccgtatcgtagttatctacacgacggggagtcaggcaactatggatgaacgaaatagacagatcgctgagataggtgcctcactgattaagcattggtaactgtcagaccaagtttactcatatatactttagattgatttaaaacttcatttttaatttaaaaggatctaggatgctgcttgcaaacaaaaaaaccaccgctaccagcggtggtttgtttgccggatcaagagctaccaactctttttccgaaggtaactggcttcagcagagcgcagataccaaatactgtccttctagtgtagccgtagttaggccaccacttcaagaactctgtagcaccgcctacatacctcgctctgctaatcctgttaccagtggctgctgccagtggcgataagtcgtgtcttaccgggttggactcaagacgatagttaccggataaggcgcagcggtcgggctgaacggggggttcgtgcacacagcccagcttggagcgaacgacctacaccgaactgagatacctacagcgtgagctatgagaaagcgccacgcttcccgaagggagaaaggcggacaggtatccggtaagcggcagggtcggaacaggagagcgcacgagggagcttccagggggaaacgcctggtatctttatagtcctgtcgggtttcgccacctctgacttgagcgtcgatttttgtgatgctcgtcaggggggcggagcctatggaaaaacgccagcaacggagatgcgccgcgtgcggctgctggagatggcggacgcgatggatatgttctgccaagggttggtttgcgcattcacagttctccgcaagaattgattggctccaattcttggagtggtgaatccgttagcgaggtgccgccggcttccattcaggtcgaggtggcccggctccatgcaccgcgacgcaacgcggggaggcagacaaggtatagggcggcgcctacaatccatgccaacccgttccatgtgctcgccgaggcggcataaatcgccgtgacgatcagcggtccaatgatcgaagttaggctggtaagagccgcgagcgatccttgaagctgtccctgatggtcgtcatctacctgcctggacagcatggcctgcaacgcgggcatcccgatgccgccggaagcgagaagaatcataatggggaaggccatccagcctcgcgtcggggagctttttgcaaaagcctaggcctccaaaaaagcctcctcactacttctggaatagctcagaggccgaggcggcctcggcctctgcataaataaaaaaaattagtcagccatgagcttggcccattgcatacgttgtatccatatcataatatgtacatttatattggctcatgtccaacattaccgccatgttgacattgattattg

SEQ ID NO: 5 - DNA, 10092 bp, Artificial Sequence
  expression cassette for CMV.SpCas9.P2A. EGFP.2xTS.gPRE.pA
  promoter 1..589: /note="human CMV immediate early promoter"
  misc_feature 1..6945: /note="expression cassette for CMV.SpCas9.P2A. EGFP.2xTS.gPRE.pA"
  TATA_signal 554..560: /note="TATA box"
  misc_feature 583: /note="transcription start point"
  CDS 612..4838: /gene="SpCas9 gene editing nuclease" /transl_table=1
  CDS 615..638: /note="FLAG tag" /transl_table=1
  CDS 645..665: /note="SV40 NLS" /transl_table=1
  CDS 4791..4838: /note="nucleoplasmin NLS" /transl_table=1
  CDS 4845..4910: /function="Porcine Teschovirus 2 A (P2A)" /transl_table=1
  CDS 4911..5630: /gene="EGFP" /transl_table=1
  protein_bind 5666..5799: /function="MS2 target site (2x TS)"
  protein_bind 5697..5719: /function="target site (TS) hairpin"
  protein_bind 5736..5758: /function="target site (TS) hairpin"
  misc_feature 5800..6701: /note="PRE"
  polyA_signal 6911..6916: /note="SV40 early mRNA polyadenylation signal"
  misc_feature 6940..6945: /note="SV40 early mRNA polyadenylation signal"
  misc_feature 7008..7463: /note="F1 single-strand DNA origin (in antisense orientation)"
  promoter 7525..7553: /note="bacterial beta-lactamase promoter for expressing kanamycin resistance gene"
  promoter 7637..7866: /note="SV40 early promoter, overlapping with SV40 ori at nt7553"
  misc_feature 7804..7939: /note="SV40 origin of replication"
  CDS 7988..8782: /gene="kanamycin/neomycin resistance" /transl_table=1
  polyA_signal 9014..9060: /note="HSV thymidine kinase (TK) polyadenylation signal"
  misc_feature 9367..10010: /note="pUC plasmid origin of replication"
tagttattaatagtaatcaattacggggtcattagttcatagcccatatatggagttccgcgttacataacttacggtaaatggcccgcctggctgaccgcccaacgacccccgcccattgacgtcaataatgacgtatgttcccatagtaacgccaatagggactttccattgacgtcaatgggtggagtatttacggtaaactgcccacttggcagtacatcaagtgtatcatatgccaagtacgccccctattgacgtcaatgacggtaaatggcccgcctggcattatgcccagtacatgaccttatgggactttcctacttggcagtacatctacgtattagtcatcgctattaccatggtgatgcggttttggcagtacatcaatgggcgtggatagcggtttgactcacggggatttccaagtctccaccccattgacgtcaatgggagtttgttttggcaccaaaatcaacgggactttccaaaatgtcgtaacaactccgccccattgacgcaaatgggcggtaggcgtgtacggtgggaggtctatataagcagagctggtttagtgaaccgtcagatccgctagcgctaccggtgccaccatggattacaaagacgatgacgataagatggccccaaagaagaagcggaaggtcggtatccacggagtcccagcagccgacaagaagtacagcatcggcctggacatcggcaccaactctgtgggctgggccgtgatcaccgacgagtacaaggtgcccagcaagaaattcaaggtgctgggcaacaccgaccggcacagcatcaagaagaacctgatcggagccctgctgttcgacagcggcgaaacagccgaggccacccggctgaagagaaccgccagaagaagatacaccagacggaagaaccggatctgctatctgcaagagatcttcagcaacgagatggccaaggtggacgacagcttcttccacagactggaagagtccttcctggtggaagaggataagaagcacgagcggcaccccatcttcggcaacatcgtggacgaggtggcctaccacgagaagtaccccaccatctaccacctgagaaagaaactggtggacagcaccgacaaggccgacctgcggctgatctatctggccctggcccacatgatcaagttccggggccacttcctgatcgagggcgacctgaaccccgacaacagcgacgtggacaagctgttcatccagctggtgcagacctacaaccagctgttcgaggaaaaccccatcaacgccagcggcgtggacgccaaggccatcctgtctgccagactgagcaagagcagacggctggaaaatctgatcgcccagctgcccggcgagaagaagaatggcctgttcggcaacctgattgccctgagcctgggcctgacccccaacttcaagagcaacttcgacctggccgaggatgccaaactgcagctgagcaaggacacctacgacgacgacctggacaacctgctggcccagatcggcgaccagtacgccgacctgtttctggccgccaagaacctgtccgacgccatcctgctgagcgacatcctgagagtgaacaccgagatcaccaaggcccccctgagcgcctctatgatcaagagatacgacgagcaccaccaggacctgaccctgctgaaagctctcgtgcggcagcagctgcctgagaagtacaaagagattttcttcgaccagagcaagaacggctacgccggctacattgacggcggagccagccaggaagagttctacaagttcatcaagcccatcctggaaaagatggacggcaccgaggaactgctcgtgaagctgaacagagaggacctgctgcggaagcagcggaccttcgacaacggcagcatcccccaccagatccacctgggagagctgcacgccattctgcggcggcaggaagatttttacccattcctgaaggacaaccgggaaaagatcgagaagatcctgaccttccgcatcccctactacgtgggccctctggccaggggaaacagcagattcgcctggatgaccagaaagagcgaggaaaccatcaccccctggaacttcgaggaagtggtggacaagggcgcttccgcccagagcttcatcgagcggatgaccaacttcgataagaacctgcccaacgagaaggtgctgcccaagcacagcctgctgtacgagtacttcaccgtgtataacgagctgaccaaagtgaaatacgtgaccgagggaatgagaaagcccgccttcctgagcggcgagcagaaaaaggccatcgtggacctgctgttcaagaccaaccggaaagtgaccgtgaagcagctgaaagaggactacttcaagaaaatcgagtgcttcgactccgtggaaatctccggcgtggaagatcggttcaacgcctccctgggcacataccacgatctgctgaaaattatcaaggacaaggacttcctggacaatgaggaaaacgaggacattctggaagatatcgtgctgaccctgacactgtttgaggacagagagatgatcgaggaacggctgaaaacctatgcccacctgttcgacgacaaagtgatgaagcagctgaagcggcggagatacaccggctggggcaggctgagccggaagctgatcaacggcatccgggacaagcagtccggcaagacaatcctggatttcctgaagtccgacggcttcgccaacagaaacttcatgcagctgatccacgacgacagcctgacctttaaagaggacatccagaaagcccaggtgtccggccagggcgatagcctgcacgagcacattgccaatctggccggcagccccgccattaagaagggcatcctgcagacagtgaaggtggtggacgagctcgtgaaagtgatgggccggcacaagcccgagaacatcgtgatcgaaatggccagagagaaccagaccacccagaagggacagaagaacagccgcgagagaatgaagcggatcgaagagggcatcaaagagctgggcagccagatcctgaaagaacaccccgtggaaaacacccagctgcagaacgagaagctgtacctgtactacctgcagaatgggcgggatatgtacgtggaccaggaactggacatcaaccggctgtccgactacgatgtggaccatatcgtgcctcagagctttctgaaggacgactccatcgacaacaaggtgctgaccagaagcgacaagaaccggggcaagagcgacaacgtgccctccgaagaggtcgtgaagaagatgaagaactactggcggcagctgctgaacgccaagctgattacccagagaaagttcgacaatctgaccaaggccgagagaggcggcctgagcgaactggataaggccggcttcatcaagagacagctggtggaaacccggcagatcacaaagcacgtggcacagatcctggactcccggatgaacactaagtacgacgagaatgacaagctgatccgggaagtgaaagtgatcaccctgaagtccaagctggtgtccgatttccggaaggatttccagttttacaaagtgcgcgagatcaacaactaccaccacgcccacgacgcctacctgaacgccgtcgtgggaaccgccctgatcaaaaagtaccctaagctggaaagcgagttcgtgtacggcgactacaaggtgtacgacgtgcggaagatgatcgccaagagcgagcaggaaatcggcaaggctaccgccaagtacttcttctacagcaacatcatgaactttttcaagaccgagattaccctggccaacggcgagatccggaagcggcctctgatcgagacaaacggcgaaaccggggagatcgtgtgggataagggccgggattttgccaccgtgcggaaagtgctgagcatgccccaagtgaatatcgtgaaaaagaccgaggtgcagacaggcggcttcagcaaagagtctatcctgcccaagaggaacagcgataagctgatcgccagaaagaaggactgggaccctaagaagtacggcggcttcgacagccccaccgtggcctattctgtgctggtggtggccaaagtggaaaagggcaagtccaagaaactgaagagtgtgaaagagctgctggggatcaccatcatggaaagaagcagcttcgagaagaatcccatcgactttctggaagccaagggctacaaagaagtgaaaaaggacctgatcatcaagctgcctaagtactccctgttcgagctggaaaacggccggaagagaatgctggcctctgccggcgaactgcagaagggaaacgaactggccctgccctccaaatatgtgaacttcctgtacctggccagccactatgagaagctgaagggctcccccgaggataatgagcagaaacagctgtttgtggaacagcacaagcactacctggacgagatcatcgagcagatcagcgagttctccaagagagtgatcctggccgacgctaatctggacaaagtgctgtccgcctacaacaagcaccgggataagcccatcagagagcaggccgagaatatcatccacctgtttaccctgaccaatctgggagcccctgccgccttcaagtactttgacaccaccatcgaccggaagaggtacaccagcaccaaagaggtgctggacgccaccctgatccaccagagcatcaccggcctgtacgagacacggatcgacctgtctcagctgggaggcgacaagcgtcctgctgctactaagaaagctggtcaagctaagaaaaagaaagctagcggcagcggcgccaccaacttcagcctgctgaagcaggccggcgacgtggaggagaaccccggccccatggtgagcaagggcgaggagctgttcaccggggtggtgcccatcctggtcgagctggacggcgacgtaaacggccacaagttcagcgtgtccggcgagggcgagggcgatgccacctacggcaagctgaccctgaagttcatctgcaccaccggcaagctgcccgtgccctggcccaccctcgtgaccaccctgacctacggcgtgcagtgcttcagccgctaccccgaccacatgaagcagcacgacttcttcaagtccgccatgcccgaaggctacgtccaggagcgcaccatcttcttcaaggacgacggcaactacaagacccgcgccgaggtgaagttcgagggcgacaccctggtgaaccgcatcgagctgaagggcatcgacttcaaggaggacggcaacatcctggggcacaagctggagtacaactacaacagccacaacgtctatatcatggccgacaagcagaagaacggcatcaaggtgaacttcaagatccgccacaacatcgaggacggcagcgtgcagctcgccgaccactaccagcagaacacccccatcggcgacggccccgtgctgctgcccgacaaccactacctgagcacccagtccgccctgagcaaagaccccaacgagaagcgcgatcacatggtcctgctggagttcgtgaccgccgccgggatcactctcggcatggacgagctgtacaagtaaagcggccgcgtcgagtttttcagcaagatgccgcctcgagagatcctaaggtacctaattgcctagaaaacatgaggatcacccatgtctgcaggtcgactctagaaaacatgaggatcacccatgtctgcagtattcccgggttcattagatcctaaggtaccgaattcgagcatcttaccgccatttattcccatatttgttctgtttttcttgatttgggtatacatttaaatgttaataaaacaaaatggtggggcaatcatttacattttatgggatatgtaattactagttcaggtgtattgccacaagacaaacatgttaagaaactttcccgttatttacgctctgttcctgttaatcaacctctggattacaaaatttgtgaaagattgactgatattcttaactatgttgctccttttacgctgtgtggatatgctgctttaatgcctctgtatcatgctattgcttcccgtacggctttcgttttctcctccttgtataaatcctggttgctgtctctttatgaggagttgtggcccgttgtccgtcaacgtggcgtggtgtgctctgtgtttgctgacgcaacccccactggctggggcattgccaccacctgtcaactcctttctgggactttcgctttccccctcccgatcgccacggcagaactcatcgccgcctgccttgcccgctgctggacaggggctaggttgctgggcactgataattccgtggtgttgtcggggaagctgacgtcctttccatggctgctcgcctgtgttgccaactggatcctgcgcgggacgtccttctgctacgtcccttcggctctcaatccagcggacctcccttcccgaggccttctgccggttctgcggcctctcccgcgtcttcgctttcggcctccgacgagtcggatctccctttgggccgcctccccgcctgtttcgcctcggcgtccggtccgtgttgcttggtcgtcacctgtgcagaattgcgaaccatggattccaccgtgaactttgtctcctggcatgcaaatcgtcaacttggcatgccaagaattcggatccaagcttcgaattctgcagtcgacggtaccgcgggcccgggatccaccggatctagataactgatcataatcagccataccacatttgtagaggttttacttgctttaaaaaacctcccacacctccccctgaacctgaaacataaaatgaatgcaattgttgttgttaacttgtttattgcagcttataatggttacaaataaagcaatagcatcacaaatttcacaaataaagcatttttttcactgcattctagttgtggtttgtccaaactcatcaatgtatcttaacgcgtaaattgtaagcgttaatattttgttaaaattcgcgttaaatttttgttaaatcagctcattttttaaccaataggccgaaatcggcaaaatcccttataaatcaaaagaatagaccgagatagggttgagtgttgttccagtttggaacaagagtccactattaaagaacgtggactccaacgtcaaagggcgaaaaaccgtctatcagggcgatggcccactacgtgaaccatcaccctaatcaagttttttggggtcgaggtgccgtaaagcactaaatcggaaccctaaagggagcccccgatttagagcttgacggggaaagccggcgaacgtggcgagaaaggaagggaagaaagcgaaaggagcgggcgctagggcgctggcaagtgtagcggtcacgctgcgcgtaaccaccacacccgccgcgcttaatgcgccgctacagggcgcgtcaggtggcacttttcggggaaatgtgcgcggaacccctatttgtttatttttctaaatacattcaaatatgtatccgctcatgagacaataaccctgataaatgcttcaataatattgaaaaaggaagagtcctgaggcggaaagaaccagctgtggaatgtgtgtcagttagggtgtggaaagtccccaggctccccagcaggcagaagtatgcaaagcatgcatctcaattagtcagcaaccaggtgtggaaagtccccaggctccccagcaggcagaagtatgcaaagcatgcatctcaattagtcagcaaccatagtcccgcccctaactccgcccatcccgcccctaactccgcccagttccgcccattctccgccccatggctgactaattttttttatttatgcagaggccgaggccgcctcggcctctgagctattccagaagtagtgaggaggcttttttggaggcctaggcttttgcaaagatcgatcaagagacaggatgaggatcgtttcgcatgattgaacaagatggattgcacgcaggttctccggccgcttgggtggagaggctattcggctatgactgggcacaacagacaatcggctgctctgatgccgccgtgttccggctgtcagcgcaggggcgcccggttctttttgtcaagaccgacctgtccggtgccctgaatgaactgcaagacgaggcagcgcggctatcgtggctggccacgacgggcgttccttgcgcagctgtgctcgacgttgtcactgaagcgggaagggactggctgctattgggcgaagtgccggggcaggatctcctgtcatctcaccttgctcctgccgagaaagtatccatcatggctgatgcaatgcggcggctgcatacgcttgatccggctacctgcccattcgaccaccaagcgaaacatcgcatcgagcgagcacgtactcggatggaagccggtcttgtcgatcaggatgatctggacgaagagcatcaggggctcgcgccagccgaactgttcgccaggctcaaggcgagcatgcccgacggcgaggatctcgtcgtgacccatggcgatgcctgcttgccgaatatcatggtggaaaatggccgcttttctggattcatcgactgtggccggctgggtgtggcggaccgctatcaggacatagcgttggctacccgtgatattgctgaagagcttggcggcgaatgggctgaccgcttcctcgtgctttacggtatcgccgctcccgattcgcagcgcatcgccttctatcgccttcttgacgagttcttctgagcgggactctggggttcgaaatgaccgaccaagcgacgcccaacctgccatcacgagatttcgattccaccgccgccttctatgaaaggttgggcttcggaatcgttttccgggacgccggctggatgatcctccagcgcggggatctcatgctggagttcttcgcccaccctagggggaggctaactgaaacacggaaggagacaataccggaaggaacccgcgctatgacggcaataaaaagacagaataaaacgcacggtgttgggtcgtttgttcataaacgcggggttcggtcccagggctggcactctgtcgataccccaccgagaccccattggggccaatacgcccgcgtttcttccttttccccaccccaccccccaagttcgggtgaaggcccagggctcgcagccaacgtcggggcggcaggccctgccatagcctcaggttactcatatatactttagattgatttaaaacttcatttttaatttaaaaggatctaggtgaagatcctttttgataatctcatgaccaaaatcccttaacgtgagttttcgttccactgagcgtcagaccccgtagaaaagatcaaaggatcttcttgagatcctttttttctgcgcgtaatctgctgcttgcaaacaaaaaaaccaccgctaccagcggtggtttgtttgccggatcaagagctaccaactctttttccgaaggtaactggcttcagcagagcgcagataccaaatactgtccttctagtgtagccgtagttaggccaccacttcaagaactctgtagcaccgcctacatacctcgctctgctaatcctgttaccagtggctgctgccagtggcgataagtcgtgtcttaccgggttggactcaagacgatagttaccggataaggcgcagcggtcgggctgaacggggggttcgtgcacacagcccagcttggagcgaacgacctacaccgaactgagatacctacagcgtgagctatgagaaagcgccacgcttcccgaagggagaaaggcggacaggtatccggtaagcggcagggtcggaacaggagagcgcacgagggagcttccagggggaaacgcctggtatctttatagtcctgtcgggtttcgccacctctgacttgagcgtcgatttttgtgatgctcgtcaggggggcggagcctatggaaaaacgccagcaacgcggcctttttacggttcctggccttttgctggccttttgctcacatgttctttcctgcgttatcccctgattctgtggataaccgtattaccgccatgcat

SEQ ID NO: 6 - DNA, 6732 bp, Artificial Sequence
  CMV.FireFly.2xTS.gPRE.pA expression cassette
  promoter 1..589: /note="human CMV immediate early promoter"
  enhancer 59..465: /note="enhancer region"
  TATA_signal 554..560: /note="TATA box"
  misc_feature 583: /note="transcription start point"
  CDS 624..2276: /gene="firefly luciferase" /transl_table=1
  protein_bind 2306..2439: /note="MS2 target site fragment (2x TS)"
  protein_bind 2337..2359: /function="target site (TS) hairpin"
  protein_bind 2376..2398: /function="target site (TS) hairpin"
  misc_feature 2440..3342: /function="PRE"
  polyA_signal 3519..3524: /note="SV40 mRNA polyadenylation signal"
  polyA_signal 3548..3553: /note="SV40 mRNA polyadenylation signal"
  misc_feature 3616..4071: /note="F1 single-strand DNA origin in antisense orientation"
  promoter 4133..4161: /note="bacterial beta-lactamase promoter for expressing kanamycin gene"
  misc_feature 4412..4547: /note="SV40 origin of replicatin"
  gene 4596..5390: /note="kanamycin/neomycin resistance"
  polyA_signal 5622..5668: /note="HSV thymidine kinase (TK) polyadenylation signal"
  misc_feature 5975..6618: /note="pUC plasmid origin of replication"
tagttattaatagtaatcaattacggggtcattagttcatagcccatatatggagttccgcgttacataacttacggtaaatggcccgcctggctgaccgcccaacgacccccgcccattgacgtcaataatgacgtatgttcccatagtaacgccaatagggactttccattgacgtcaatgggtggagtatttacggtaaactgcccacttggcagtacatcaagtgtatcatatgccaagtacgccccctattgacgtcaatgacggtaaatggcccgcctggcattatgcccagtacatgaccttatgggactttcctacttggcagtacatctacgtattagtcatcgctattaccatggtgatgcggttttggcagtacatcaatgggcgtggatagcggtttgactcacggggatttccaagtctccaccccattgacgtcaatgggagtttgttttggcaccaaaatcaacgggactttccaaaatgtcgtaacaactccgccccattgacgcaaatgggcggtaggcgtgtacggtgggaggtctatataagcagagctggtttagtgaaccgtcagatccgctagcgctaccgggactgttggtaaagccaccatggaagatgccaaaaacattaagaagggcccagcgccattctacccactcgaagacgggaccgccggcgagcagctgcacaaagccatgaagcgctacgccctggtgcccggcaccatcgcctttaccgacgcacatatcgaggtggacattacctacgccgagtacttcgagatgagcgttcggctggcagaagctatgaagcgctatgggctgaatacaaaccatcggatcgtggtgtgcagcgagaatagcttgcagttcttcatgcccgtgttgggtgccctgttcatcggtgtggctgtggccccagctaacgacatctacaacgagcgcgagctgctgaacagcatgggcatcagccagcccaccgtcgtattcgtgagcaagaaagggctgcaaaagatcctcaacgtgcaaaagaagctaccgatcatacaaaagatcatcatcatggatagcaagaccgactaccagggcttccaaagcatgtacaccttcgtgacttcccatttgccacccggcttcaacgagtacgacttcgtgcccgagagcttcgaccgggacaaaaccatcgccctgatcatgaacagtagtggcagtaccggattgcccaagggcgtagccctaccgcaccgcaccgcttgtgtccgattcagtcatgcccgcgaccccatcttcggcaaccagatcatccccgacaccgctatcctcagcgtggtgccatttcaccacggcttcggcatgttcaccacgctgggctacttgatctgcggctttcgggtcgtgctcatgtaccgcttcgaggaggagctattcttgcgcagcttgcaagactataagattcaatctgccctgctggtgcccacactatttagcttcttcgctaagagcactctcatcgacaagtacgacctaagcaacttgcacgagatcgccagcggcggggcgccgctcagcaaggaggtaggtgaggccgtggccaaacgcttccacctaccaggcatccgccagggctacggcctgacagaaacaaccagcgccattctgatcacccccgaaggggacgacaagcctggcgcagtaggcaaggtggtgcccttcttcgaggctaaggtggtggacttggacaccggtaagacactgggtgtgaaccagcgcggcgagctgtgcgtccgtggccccatgatcatgagcggctacgttaacaaccccgaggctacaaacgctctcatcgacaaggacggctggctgcacagcggcgacatcgcctactgggacgaggacgagcacttcttcatcgtggaccggctgaagagcctgatcaaatacaagggctaccaggtagccccagccgaactggagagcatcctgctgcaacaccccaacatcttcgacgccggggtcgccggcctgcccgacgacgatgccggcgagctgcccgccgcagtcgtcgtgctggaacacggtaaaaccatgaccgagaaggagatcgtggactatgtggccagccaggttacaaccgccaagaagctgcgcggtggtgttgtgttcgtggacgaggtgcctaaaggactgaccggcaagttggacgcccgcaagatccgcgagattctcattaaggccaagaagggcggcaagatcgccgtgtaataattctagagtcggggcggccggccgcgtcgagagatcctaaggtacctaattgcctagaaaacatgaggatcacccatgtctgcaggtcgactctagaaaacatgaggatcacccatgtctgcagtattcccgggttcattagatcctaaggtaccgaattcgagcatcttaccgccatttattcccatatttgttctgtttttcttgatttgggtatacatttaaatgttaataaaacaaaatggtggggcaatcatttacattttatgggatatgtaattactagttcaggtgtattgccacaagacaaacatgttaagaaactttcccgttatttacgctctgttcctgttaatcaacctctggattacaaaatttgtgaaagattgactgatattcttaactatgttgctccttttacgctgtgtggatatgctgctttaatgcctctgtatcatgctattgcttcccgtacggctttcgttttctcctccttgtataaatcctggttgctgtctctttatgaggagttgtggcccgttgtccgtcaacgtggcgtggtgtgctctgtgtttgctgacgcaacccccactggctggggcattgccaccacctgtcaactcctttctgggactttcgctttccccctcccgatcgccacggcagaactcatcgccgcctgccttgcccgctgctggacaggggctaggttgctgggcactgataattccgtggtgttgtcggggaagctgacgtcctttccatggctgctcgcctgtgttgccaactggatcctgcgcgggacgtccttctgctacgtcccttcggctctcaatccagcggacctcccttcccgaggccttctgccggttctgcggcctctcccgcgtcttcgctttcggcctccgacgagtcggatctccctttgggccgcctccccgcctgtttcgcctcggcgtccggtccgtgttgcttggtcgtcacctgtgcagaattgcgaaccatggattccaccgtgaactttgtctcctggcatgcaaatcgtcaacttggcatgccaagaattcggatccaagcttcgaattctgcagtcgacggtaccgcgggcccgggatccaccggatctagataactgatcataatcagccataccacatttgtagaggttttacttgctttaaaaaacctcccacacctccccctgaacctgaaacataaaatgaatgcaattgttgttgttaacttgtttattgcagcttataatggttacaaataaagcaatagcatcacaaatttcacaaataaagcatttttttcactgcattctagttgtggtttgtccaaactcatcaatgtatcttaacgcgtaaattgtaagcgttaatattttgttaaaattcgcgttaaatttttgttaaatcagctcattttttaaccaataggccgaaatcggcaaaatcccttataaatcaaaagaatagaccgagatagggttgagtgttgttccagtttggaacaagagtccactattaaagaacgtggactccaacgtcaaagggcgaaaaaccgtctatcagggcgatggcccactacgtgaaccatcaccctaatcaagttttttggggtcgaggtgccgtaaagcactaaatcggaaccctaaagggagcccccgatttagagcttgacggggaaagccggcgaacgtggcgagaaaggaagggaagaaagcgaaaggagcgggcgctagggcgctggcaagtgtagcggtcacgctgcgcgtaaccaccacacccgccgcgcttaatgcgccgctacagggcgcgtcaggtggcacttttcggggaaatgtgcgcggaacccctatttgtttatttttctaaatacattcaaatatgtatccgctcatgagacaataaccctgataaatgcttcaataatattgaaaaaggaagagtcctgaggcggaaagaaccagctgtggaatgtgtgtcagttagggtgtggaaagtccccaggctccccagcaggcagaagtatgcaaagcatgcatctcaattagtcagcaaccaggtgtggaaagtccccaggctccccagcaggcagaagtatgcaaagcatgcatctcaattagtcagcaaccatagtcccgcccctaactccgcccatcccgcccctaactccgcccagttccgcccattctccgccccatggctgactaattttttttatttatgcagaggccgaggccgcctcggcctctgagctattccagaagtagtgaggaggcttttttggaggcctaggcttttgcaaagatcgatcaagagacaggatgaggatcgtttcgcatgattgaacaagatggattgcacgcaggttctccggccgcttgggtggagaggctattcggctatgactgggcacaacagacaatcggctgctctgatgccgccgtgttccggctgtcagcgcaggggcgcccggttctttttgtcaagaccgacctgtccggtgccctgaatgaactgcaagacgaggcagcgcggctatcgtggctggccacgacgggcgttccttgcgcagctgtgctcgacgttgtcactgaagcgggaagggactggctgctattgggcgaagtgccggggcaggatctcctgtcatctcaccttgctcctgccgagaaagtatccatcatggctgatgcaatgcggcggctgcatacgcttgatccggctacctgcccattcgaccaccaagcgaaacatcgcatcgagcgagcacgtactcggatggaagccggtcttgtcgatcaggatgatctggacgaagagcatcaggggctcgcgccagccgaactgttcgccaggctcaaggcgagcatgcccgacggcgaggatctcgtcgtgacccatggcgatgcctgcttgccgaatatcatggtggaaaatggccgcttttctggattcatcgactgtggccggctgggtgtggcggaccgctatcaggacatagcgttggctacccgtgatattgctgaagagcttggcggcgaatgggctgaccgcttcctcgtgctttacggtatcgccgctcccgattcgcagcgcatcgccttctatcgccttcttgacgagttcttctgagcgggactctggggttcgaaatgaccgaccaagcgacgcccaacctgccatcacgagatttcgattccaccgccgccttctatgaaaggttgggcttcggaatcgttttccgggacgccggctggatgatcctccagcgcggggatctcatgctggagttcttcgcccaccctagggggaggctaactgaaacacggaaggagacaataccggaaggaacccgcgctatgacggcaataaaaagacagaataaaacgcacggtgttgggtcgtttgttcataaacgcggggttcggtcccagggctggcactctgtcgataccccaccgagaccccattggggccaatacgcccgcgtttcttccttttccccaccccaccccccaagttcgggtgaaggcccagggctcgcagccaacgtcggggcggcaggccctgccatagcctcaggttactcatatatactttagattgatttaaaacttcatttttaatttaaaaggatctaggtgaagatcctttttgataatctcatgaccaaaatcccttaacgtgagttttcgttccactgagcgtcagaccccgtagaaaagatcaaaggatcttcttgagatcctttttttctgcgcgtaatctgctgcttgcaaacaaaaaaaccaccgctaccagcggtggtttgtttgccggatcaagagctaccaactctttttccgaaggtaactggcttcagcagagcgcagataccaaatactgtccttctagtgtagccgtagttaggccaccacttcaagaactctgtagcaccgcctacatacctcgctctgctaatcctgttaccagtggctgctgccagtggcgataagtcgtgtcttaccgggttggactcaagacgatagttaccggataaggcgcagcggtcgggctgaacggggggttcgtgcacacagcccagcttggagcgaacgacctacaccgaactgagatacctacagcgtgagctatgagaaagcgccacgcttcccgaagggagaaaggcggacaggtatccggtaagcggcagggtcggaacaggagagcgcacgagggagcttccagggggaaacgcctggtatctttatagtcctgtcgggtttcgccacctctgacttgagcgtcgatttttgtgatgctcgtcaggggggcggagcctatggaaaaacgccagcaacgcggcctttttacggttcctggccttttgctggccttttgctcacatgttctttcctgcgttatcccctgattctgtggataaccgtattaccgccatgcat

SEQ ID NO: 7 - DNA, 20 bp, Artificial Sequence
  sgRNA for targeting mouse methylcytosine dioxygenase Tet2
gaacaagctctacatcccgt

SEQ ID NO: 8 - DNA, 21 bp, Artificial Sequence
  sgRNA targeting mouse cellular tumor antigen p53
gaggagctcctgacactcgga

SEQ ID NO: 9 - DNA, 20 bp, Artificial Sequence
  sgRNA for targeting human cellular tumor antigen p53
gacggaaaccgtagctgccc

SEQ ID NO: 10 - DNA, 20 bp, Artificial Sequence
  sgRNA for targeting human C-X-C chemokine receptor 4
gttccagtttcagcacatca

SEQ ID NO: 11 - DNA, 20 bp, Artificial Sequence
  sgRNA for targeting enhanced green fluorescent protein
gcactgcacgccgtaggtca

SEQ ID NO: 12 - DNA, 8868 bp, Artificial Sequence
  CMV.ASLV.gag.co.PR.pr.MS2.pA
  promoter 232..819: /note="human CMV immediate early promoter"
  intron 907..1450: /note="beta-globin intron"
  CDS 1462..1914: /note="MA matrix" /transl_table=1
  CDS 1915..1935: /note="protease site" /transl_table=1
  CDS 1936..1986: /note="p2" /transl_table=1
  CDS 1987..2007: /note="protease site" /transl_table=1
  CDS 2008..2172: /note="p10" /transl_table=1
  CDS 2173..2193: /note="protease site" /transl_table=1
  CDS 2194..2919: /note="CA capsid" /transl_table=1
  CDS 2920..2940: /note="protease site" /transl_table=1
  CDS 2941..3186: /note="NC nucleocapsid" /transl_table=1
  CDS 3187..3207: /note="protease site" /transl_table=1
  CDS 3208..3573: /note="PR protease" /transl_table=1
  CDS 3574..3594: /note="protease site" /transl_table=1
  CDS 3595..3612: /note="glycin linker" /transl_table=1
  CDS 3613..4002: /note="MS2CP" /transl_table=1
  CDS 3613..4389: /note="MS2 coat protein dimer (2xMS2CP)" /transl_table=1
  misc_feature 4003..4005: /note="Alanin linker"
  CDS 4006..4389: /note="MS2CP" /transl_table=1
  polyA_signal 4468..4692: /note="bgH polyA signal"
  misc_feature 4738..5166: /note="F1 ori"
  promoter 5180..5509: /note="SV40 promoter"
  gene 5576..6370: /note="Kanamycin/Neomycin resistance gene"
  polyA_signal 6544..6665: /note="SV40 polyA signal"
  misc_feature 7116..7701: /note="ori"
  gene 7872..8732: /note="Ampicillin resistance gene in antisense orientation"
  misc_feature 8774..8802: /note="Ampicillin resistance gene promoter in antisense orientation"
gacggatcgggagatctcccgatcccctatggtgcactctcagtacaatctgctctgatgccgcatagttaagccagtatctgctccctgcttgtgtgttggaggtcgctgagtagtgcgcgagcaaaatttaagctacaacaaggcaaggcttgaccgacaattgcatgaagaatctgcttagggttaggcgttttgcgctgcttcgcgatgtacgggccagatatacgcgttgacattgattattgactagttattaatagtaatcaattacggggtcattagttcatagcccatatatggagttccgcgttacataacttacggtaaatggcccgcctggctgaccgcccaacgacccccgcccattgacgtcaataatgacgtatgttcccatagtaacgccaatagggactttccattgacgtcaatgggtggactatttacggtaaactgcccacttggcagtacatcaagtgtatcatatgccaagtacgccccctattgacgtcaatgacggtaaatggcccgcctggcattatgcccagtacatgaccttatgggactttcctacttggcagtacatctacgtattagtcatcgctattaccatggtgatgcggttttggcagtacatcaatgggcgtggatagcggtttgactcacggggatttccaagtctccaccccattgacgtcaatgggagtttgttttggcaccaaaatcaacgggactttccaaaatgtcgtaacaactccgccccattgacgcaaatgggcggtaggcgtgtacggtgggaggtctatataagcagagctctctggctaactagagaacccactgcttactggcttatcgaaattaatacgactcactatagggagacccaagcttggtaccgagctcggatcctgagaacttcagggtgagtctatgggacccttgatgttttctttccccttcttttctatggttaagttcatgtcataggaaggggagaagtaacagggtacacatattgaccaaatcagggtaattttgcatttgtaattttaaaaaatgctttcttcttttaatatacttttttgtttatcttatttctaatactttccctaatctctttctttcagggcaataatgatacaatgtatcatgcctctttgcaccattctaaagaataacagtgataatttctgggttaaggcaatagcaatatttctgcatataaatatttctgcatataaattgtaactgatgtaagaggtttcatattgctaatagcagctacaatccagctaccattctgcttttattttatggttgggataaggctggattattctgagtccaagctaggcccttttgctaatcatgttcatacctcttatcttcctcccacagctcctgggcaacgtgctggtctgtgtgctggcccatcactttggcaaagaattcgccaccatggaagccgtgatcaaagtgatcagcagcgcctgcaagacctactgcggcaagatcagccccagcaagaaagaaatcggcgctatgctgtctctcctgcaaaaggaaggcctgctgatgagccccagcgacctgtacagccccggcagctgggatcctatcacagccgccctgagccagagggccatggtgctgggcaagagcggcgagctgaaaacctgggggctggtgctgggagccctgaaggccgccagagaagaacaggtgaccagcgagcaggccaagttttggctgggcctgggcggaggaagagtgtctccccctggccccgagtgtatcgagaagcccgccaccgagcggagaatcgacaagggcgaggaagtgggcgagacaaccgtgcagcgggacgccaagatggcccctgaggaagccgccacccctaagaccgtgggcaccagctgctaccactgtggcaccgccgtgggctgtaattgtgccaccgccaccgcctctgcccctcctcctccttacgtgggcagcggcctgtatccttctctggccggcgtgggcgagcagcagggacagggcgacaataccagcagaggcgccgagcagcctagagaggaacctggacacgctggccaggccccaggacctgccctgacagattgggccagagtgcgggaggaactggcctctaccggaccccctgtggtggccatgcccgtggtgatcaagacagagggccctgcctggacccctctggaacccaagctgatcacccggctggccgatacagtgcggaccaagggcctgagaagccccatcaccatggccgaggtggaggccctgatgagcagccccctgctgccccacgacgtgaccaacctgatgagagtgatcctgggccctgctccctacgccctgtggatggatgcctggggcgtgcagctgcagacagtgatcgccgctgccaccagagatcccagacaccccgccaatggccagggcagaggcgagcggaccaacctggacagactgaagggcctggccgacggcatggtgggcaatcctcagggacaggccgctctgctgaggcctggcgaactggtggccatcacagccagcgccctgcaggccttcagagaggtggccagactggccgagcctgccggcccttgggccgatatcacccagggccccagcgagagcttcgtggacttcgccaaccggctgatcaaggccgtggagggcagcgatctgcctcctagcgccagagcccccgtgatcatcgactgcttccggcagaagtcccagcccgacatccagcagctgatcagagccgcccctagcaccctgaccacccctggcgagatcatcaaatacgtgctggaccggcagaagatcgcccctctgaccgatcagggcattgccgccgctatgagcagcgccatccagcctctggtgatggccgtggtgaacagagagagggacggccagacaggatctggcggcagagccagaggcctgtgctacacctgtggcagccctggccactaccaggcccagtgccccaagaagcggaagtccggcaacagccgggagagatgccagctgtgtgacggcatgggccacaacgccaagcagtgccggaagcgggatggcaatcagggccagaggcccggcagaggactgtctagcggcccttggcctggacctgagcagcctgccgtgagcctggccatgaccatggaacacaaggaccggcccctggtgcgcgtgatcctgaccaacaccggcagccaccccgtgaagcagcggagcgtgtacatcaccgccctgctggacagcggagccgacatcaccatcatcagcgaagaggactggcccaccgactggcctgtggtggacaccgccaacccccagatccacggcatcggcggaggaatccccatgcggaagtcccgggatatgatagaggtgggggttattaaccgagacgggtcgttggagcgacccctgctcctcttccccgcagtcgctatggttagagggagtatcctaggaagagattgtctgcagggcctagggctccgcttgaccaacctcagggccactgttcttactgttgcgctaaccggtggcggcggcatggcctccaacttcacccagttcgtgctggtggacaacggcggcacaggcgacgtgacagtggctcccagcaacttcgctaacggcgtggccgagtggatcagcagcaacagcagatcccaggcctacaaagtgacctgcagcgtgcggcagagcagcgcccagaaccggaagtacaccatcaaggtggaagtgcccaaggtggcaacccagacagtgggcggagtggaactgcctgtggccgcttggagaagctacctgaacatggaactgaccatccccatcttcgccaccaacagcgactgcgagctgatcgtgaaggccatgcagggcctgctgaaggacggcaaccctatcccttctgccattgccgccaacagcggcatctacgccaatttcacacagtttgtgctggtcgacaatggcggaactggcgacgtgactgtcgccccaagcaacttcgctaacggggtcgctgaatggatcagctctaactcgcgttcacaggcttacaaagtaacctgtagcgttcgtcagagctctgcgcagaatcgcaaatacaccatcaaagtcgaggtgcctaaagtggcaacccagactgttggtggtgtagagcttcctgtagccgcatggcgttcgtacttaaatatggaactaaccattccaattttcgccacgaattccgactgcgagcttattgttaaggcaatgcaaggtctcctaaaagatggaaacccgattccctcggccatcgcggcaaactccggcatctactgagcggccgctcgagcatgcatctagagggccctattctatagtgtcacctaaatgctagagctcgctgatcagcctcgactgtgccttctagttgccagccatctgttgtttgcccctcccccgtgccttccttgaccctggaaggtgccactcccactgtcctttcctaataaaatgaggaaattgcatcgcattgtctgagtaggtgtcattctattctggggggtggggtggggcaggacagcaagggggaggattgggaagacaatagcaggcatgctggggatgcggtgggctctatggcttctgaggcggaaagaaccagctggggctctagggggtatccccacgcgccctgtagcggcgcattaagcgcggcgggtgtggtggttacgcgcagcgtgaccgctacacttgccagcgccctagcgcccgctcctttcgctttcttcccttcctttctcgccacgttcgccggctttccccgtcaagctctaaatcgggggctccctttagggttccgatttagtgctttacggcacctcgaccccaaaaaacttgattagggtgatggttcacgtagtgggccatcgccctgatagacggtttttcgccctttgacgttggagtccacgttctttaatagtggactcttgttccaaactggaacaacactcaaccctatctcggtctattcttttgatttataagggattttgccgatttcggcctattggttaaaaaatgagctgatttaacaaaaatttaacgcgaattaattctgtggaatgtgtgtcagttagggtgtggaaagtccccaggctccccagcaggcagaagtatgcaaagcatgcatctcaattagtcagcaaccaggtgtggaaagtccccaggctccccagcaggcagaagtatgcaaagcatgcatctcaattagtcagcaaccatagtcccgcccctaactccgcccatcccgcccctaactccgcccagttccgcccattctccgccccatggctgactaattttttttatttatgcagaggccgaggccgcctctgcctctgagctattccagaagtagtgaggaggcttttttggaggcctaggcttttgcaaaaagctcccgggagcttgtatatccattttcggatctgatcaagagacaggatgaggatcgtttcgcatgattgaacaagatggattgcacgcaggttctccggccgcttgggtggagaggctattcggctatgactgggcacaacagacaatcggctgctctgatgccgccgtgttccggctgtcagcgcaggggcgcccggttctttttgtcaagaccgacctgtccggtgccctgaatgaactgcaggacgaggcagcgcggctatcgtggctggccacgacgggcgttccttgcgcagctgtgctcgacgttgtcactgaagcgggaagggactggctgctattgggcgaagtgccggggcaggatctcctgtcatctcaccttgctcctgccgagaaagtatccatcatggctgatgcaatgcggcggctgcatacgcttgatccggctacctgcccattcgaccaccaagcgaaacatcgcatcgagcgagcacgtactcggatggaagccggtcttgtcgatcaggatgatctggacgaagagcatcaggggctcgcgccagccgaactgttcgccaggctcaaggcgcgcatgcccgacggcgaggatctcgtcgtgacccatggcgatgcctgcttgccgaatatcatggtggaaaatggccgcttttctggattcatcgactgtggccggctgggtgtggcggaccgctatcaggacatagcgttggctacccgtgatattgctgaagagcttggcggcgaatgggctgaccgcttcctcgtgctttacggtatcgccgctcccgattcgcagcgcatcgccttctatcgccttcttgacgagttcttctgagcgggactctggggttcgaaatgaccgaccaagcgacgcccaacctgccatcacgagatttcgattccaccgccgccttctatgaaaggttgggcttcggaatcgttttccgggacgccggctggatgatcctccagcgcggggatctcatgctggagttcttcgcccaccccaacttgtttattgcagcttataatggttacaaataaagcaatagcatcacaaatttcacaaataaagcatttttttcactgcattctagttgtggtttgtccaaactcatcaatgtatcttatcatgtctgtataccgtcgacctctagctagagcttggcgtaatcatggtcatagctgtttcctgtgtgaaattgttatccgctcacaattccacacaacatacgagccggaagcataaagtgtaaagcctggggtgcctaatgagtgagctaactcacattaattgcgttgcgctcactgcccgctttccagtcgggaaacctgtcgtgccagctgcattaatgaatcggccaacgcgcggggagaggcggtttgcgtattgggcgctcttccgcttcctcgctcactgactcgctgcgctcggtcgttcggctgcggcgagcggtatcagctcactcaaaggcggtaatacggttatccacagaatcaggggataacgcaggaaagaacatgtgagcaaaaggccagcaaaaggccaggaaccgtaaaaaggccgcgttgctggcgtttttccataggctccgcccccctgacgagcatcacaaaaatcgacgctcaagtcagaggtggcgaaacccgacaggactataaagataccaggcgtttccccctggaagctccctcgtgcgctctcctgttccgaccctgccgcttaccggatacctgtccgcctttctcccttcgggaagcgtggcgctttctcatagctcacgctgtaggtatctcagttcggtgtaggtcgttcgctccaagctgggctgtgtgcacgaaccccccgttcagcccgaccgctgcgccttatccggtaactatcgtcttgagtccaacccggtaagacacgacttatcgccactggcagcagccactggtaacaggattagcagagcgaggtatgtaggcggtgctacagagttcttgaagtggtggcctaactacggctacactagaagaacagtatttggtatctgcgctctgctgaagccagttaccttcggaaaaagagttggtagctcttgatccggcaaacaaaccaccgctggtagcggtttttttgtttgcaagcagcagattacgcgcagaaaaaaaggatctcaagaagatcctttgatcttttctacggggtctgacgctcagtggaacgaaaactcacgttaagggattttggtcatgagattatcaaaaaggatcttcacctagatccttttaaattaaaaatgaagttttaaatcaatctaaagtatatatgagtaaacttggtctgacagttaccaatgcttaatcagtgaggcacctatctcagcgatctgtctatttcgttcatccatagttgcctgactccccgtcgtgtagataactacgatacgggagggcttaccatctggccccagtgctgcaatgataccgcgagacccacgctcaccggctccagatttatcagcaataaaccagccagccggaagggccgagcgcagaagtggtcctgcaactttatccgcctccatccagtctattaattgttgccgggaagctagagtaagtagttcgccagttaatagtttgcgcaacgttgttgccattgctacaggcatcgtggtgtcacgctcgtcgtttggtatggcttcattcagctccggttcccaacgatcaaggcgagttacatgatcccccatgttgtgcaaaaaagcggttagctccttcggtcctccgatcgttgtcagaagtaagttggccgcagtgttatcactcatggttatggcagcactgcataattctcttactgtcatgccatccgtaagatgcttttctgtgactggtgagtactcaaccaagtcattctgagaatagtgtatgcggcgaccgagttgctcttgcccggcgtcaatacgggataataccgcgccacatagcagaactttaaaagtgctcatcattggaaaacgttcttcggggcgaaaactctcaaggatcttaccgctgttgagatccagttcgatgtaacccactcgtgcacccaactgatcttcagcatcttttactttcaccagcgtttctgggtgagcaaaaacaggaaggcaaaatgccgcaaaaaagggaataagggcgacacggaaatgttgaatactcatactcttcctttttcaatattattgaagcatttatcagggttattgtctcatgagcggatacatatttgaatgtatttagaaaaataaacaaataggggttccgcgcacatttccccgaaaagtgccacctgacgtc

SEQ ID NO: 13 - DNA, 8163 bp, Artificial Sequence
  pcDNA3.MLV.gag.CA.pr.MS2
  promoter 232..830: /note="CMV immediate early promoter"
  intron 907..1450: /note="beta-globin intron"
  CDS 1475..1855: /note="matrix (MA)" /transl_table=1
  CDS 1475..2917: /note="gammaretroviral mouse leukemia virus Gag domains" /transl_table=1
  misc_feature 1856..1876: /note="protease site"
  CDS 1877..2107: /note="P12" /transl_table=1
  misc_feature 2108..2128: /note="protease site"
  CDS 2129..2896: /note="Capsid (CA)" /transl_table=1
  misc_feature 2897..2917: /note="protease site"
  misc_feature 2918..2935: /note="Glycin-rich linker"
  misc_feature 2936..3325: /note="MS2 coat protein"
  CDS 2936..3712: /note="MS2 coat protein dimer" /transl_table=1
  misc_feature 3326..3328: /note="linker containing Ala"
  misc_feature 3329..3712: /note="MS2 coat protein"
  polyA_signal 3763..3987: /note="bgH poly A signal"
  misc_feature 4033..4461: /note="F1 ori"
  promoter 4475..4804: /note="SV40 promoter"
  gene 4871..5665: /note="Kanamycin/neomycin resistance gene"
  polyA_signal 5839..5960: /note="SV40 poly A signal"
  misc_feature 6411..6996: /note="ori"
  misc_feature 7167..8027: /note="ampicillin resistance in antisense orientation"
  promoter 8069..8097: /note="ampicillin resistance gene promoter in antisense orientation"
gacggatcgggagatctcccgatcccctatggtgcactctcagtacaatctgctctgatgccgcatagttaagccagtatctgctccctgcttgtgtgttggaggtcgctgagtagtgcgcgagcaaaatttaagctacaacaaggcaaggcttgaccgacaattgcatgaagaatctgcttagggttaggcgttttgcgctgcttcgcgatgtacgggccagatatacgcgttgacattgattattgactagttattaatagtaatcaattacggggtcattagttcatagcccatatatggagttccgcgttacataacttacggtaaatggcccgcctggctgaccgcccaacgacccccgcccattgacgtcaataatgacgtatgttcccatagtaacgccaatagggactttccattgacgtcaatgggtggactatttacggtaaactgcccacttggcagtacatcaagtgtatcatatgccaagtacgccccctattgacgtcaatgacggtaaatggcccgcctggcattatgcccagtacatgaccttatgggactttcctacttggcagtacatctacgtattagtcatcgctattaccatggtgatgcggttttggcagtacatcaatgggcgtggatagcggtttgactcacggggatttccaagtctccaccccattgacgtcaatgggagtttgttttggcaccaaaatcaacgggactttccaaaatgtcgtaacaactccgccccattgacgcaaatgggcggtaggcgtgtacggtgggaggtctatataagcagagctctctggctaactagagaacccactgcttactggcttatcgaaattaatacgactcactatagggagacccaagcttggtaccgagctcggatcctgagaacttcagggtgagtctatgggacccttgatgttttctttccccttcttttctatggttaagttcatgtcataggaaggggagaagtaacagggtacacatattgaccaaatcagggtaattttgcatttgtaattttaaaaaatgctttcttcttttaatatacttttttgtttatcttatttctaatactttccctaatctctttctttcagggcaataatgatacaatgtatcatgcctctttgcaccattctaaagaataacagtgataatttctgggttaaggcaatagcaatatttctgcatataaatatttctgcatataaattgtaactgatgtaagaggtttcatattgctaatagcagctacaatccagctaccattctgcttttattttatggttgggataaggctggattattctgagtccaagctaggcccttttgctaatcatgttcatacctcttatcttcctcccacagctcctgggcaacgtgctggtctgtgtgctggcccatcactttggcaaagcacgtgagatctgaattcgccaccatgggccagactgttaccactcccttaagtttgaccttaggtcactggaaagatgtcgagcggatcgctcacaaccagtcggtagatgtcaagaagagacgttgggttaccttctgctctgcagaatggccaacctttaacgtcggatggccgcgagacggcacctttaaccgagacctcatcacccaggttaagatcaaggtcttttcacctggcccgcatggacacccagaccaggtcccctacatcgtgacctgggaagccttggcttttgacccccctccctgggtcaagccctttgtacaccctaagcctccgcctcctcttcctccatccgccccgtctctcccccttgaacctcctcgttcgaccccgcctcgatcctccctttatccagccctcactccttctctaggcgccaaacctaaacctcaagttctttctgacagtggggggccgctcatcgacctacttacagaagaccccccgccttatagggacccaagaccacccccttccgacagggacggaaatggtggagaagcgacccctgcgggagaggcaccggacccctccccaatggcatctcgcctacgtgggagacgggagccccctgtggccgactccactacctcgcaggcattccccctccgcgcaggaggaaacggacagcttcaatactggccgttctcctcttctgacctttacaactggaaaaataataacccttctttttctgaagatccaggtaaactgacagctctgatcgagtctgtcctcatcacccatcagcccacctgggacgactgtcagcagctgttggggactctgctgaccggagaagaaaaacaacgggtgctcttagaggctagaaaggcggtgcggggcgatgatgggcgccccactcaactgcccaatgaagtcgatgccgcttttcccctcgagcgcccagactgggattacaccacccaggcaggtaggaaccacctagtccactatcgccagttgctcctagcgggtctccaaaacgcgggcagaagccccaccaatttggccaaggtaaaaggaataacacaagggcccaatgagtctccctcggccttcctagagagacttaaggaagcctatcgcaggtacactccttatgaccctgaggacccagggcaagaaactaatgtgtctatgtctttcatttggcagtctgccccagacattgggagaaagttagagaggttagaagatttaaaaaacaagacgcttggagatttggttagagaggcagaaaagatctttaataaacgagaaaccccggaagaaagagaggaacgtatcaggagagaaacagaggaaaaagaagaacgccgtaggacagaggatgagcagaaagagaaagaaagagatcgtaggagacatagagagatgagcaagctattggccactgtcgttaccggtggcggcggcatggcctccaacttcacccagttcgtgctggtggacaacggcggcacaggcgacgtgacagtggctcccagcaacttcgctaacggcgtggccgagtggatcagcagcaacagcagatcccaggcctacaaagtgacctgcagcgtgcggcagagcagcgcccagaaccggaagtacaccatcaaggtggaagtgcccaaggtggcaacccagacagtgggcggagtggaactgcctgtggccgcttggagaagctacctgaacatggaactgaccatccccatcttcgccaccaacagcgactgcgagctgatcgtgaaggccatgcagggcctgctgaaggacggcaaccctatcccttctgccattgccgccaacagcggcatctacgccaatttcacacagtttgtgctggtcgacaatggcggaactggcgacgtgactgtcgccccaagcaacttcgctaacggggtcgctgaatggatcagctctaactcgcgttcacaggcttacaaagtaacctgtagcgttcgtcagagctctgcgcagaatcgcaaatacaccatcaaagtcgaggtgcctaaagtggcaacccagactgttggtggtgtagagcttcctgtagccgcatggcgttcgtacttaaatatggaactaaccattccaattttcgccacgaattccgactgcgagcttattgttaaggcaatgcaaggtctcctaaaagatggaaacccgattccctcggccatcgcggcaaactccggcatctactgagcggccgctcgagtctagagggcccgtttaaacccgctgatcagcctcgactgtgccttctagttgccagccatctgttgtttgcccctcccccgtgccttccttgaccctggaaggtgccactcccactgtcctttcctaataaaatgaggaaattgcatcgcattgtctgagtaggtgtcattctattctggggggtggggtggggcaggacagcaagggggaggattgggaagacaatagcaggcatgctggggatgcggtgggctctatggcttctgaggcggaaagaaccagctggggctctagggggtatccccacgcgccctgtagcggcgcattaagcgcggcgggtgtggtggttacgcgcagcgtgaccgctacacttgccagcgccctagcgcccgctcctttcgctttcttcccttcctttctcgccacgttcgccggctttccccgtcaagctctaaatcgggggctccctttagggttccgatttagtgctttacggcacctcgaccccaaaaaacttgattagggtgatggttcacgtagtgggccatcgccctgatagacggtttttcgccctttgacgttggagtccacgttctttaatagtggactcttgttccaaactggaacaacactcaaccctatctcggtctattcttttgatttataagggattttgccgatttcggcctattggttaaaaaatgagctgatttaacaaaaatttaacgcgaattaattctgtggaatgtgtgtcagttagggtgtggaaagtccccaggctccccagcaggcagaagtatgcaaagcatgcatctcaattagtcagcaaccaggtgtggaaagtccccaggctccccagcaggcagaagtatgcaaagcatgcatctcaattagtcagcaaccatagtcccgcccctaactccgcccatcccgcccctaactccgcccagttccgcccattctccgccccatggctgactaattttttttatttatgcagaggccgaggccgcctctgcctctgagctattccagaagtagtgaggaggcttttttggaggcctaggcttttgcaaaaagctcccgggagcttgtatatccattttcggatctgatcaagagacaggatgaggatcgtttcgcatgattgaacaagatggattgcacgcaggttctccggccgcttgggtggagaggctattcggctatgactgggcacaacagacaatcggctgctctgatgccgccgtgttccggctgtcagcgcaggggcgcccggttctttttgtcaagaccgacctgtccggtgccctgaatgaactgcaggacgaggcagcgcggctatcgtggctggccacgacgggcgttccttgcgcagctgtgctcgacgttgtcactgaagcgggaagggactggctgctattgggcgaagtgccggggcaggatctcctgtcatctcaccttgctcctgccgagaaagtatccatcatggctgatgcaatgcggcggctgcatacgcttgatccggctacctgcccattcgaccaccaagcgaaacatcgcatcgagcgagcacgtactcggatggaagccggtcttgtcgatcaggatgatctggacgaagagcatcaggggctcgcgccagccgaactgttcgccaggctcaaggcgcgcatgcccgacggcgaggatctcgtcgtgacccatggcgatgcctgcttgccgaatatcatggtggaaaatggccgcttttctggattcatcgactgtggccggctgggtgtggcggaccgctatcaggacatagcgttggctacccgtgatattgctgaagagcttggcggcgaatgggctgaccgcttcctcgtgctttacggtatcgccgctcccgattcgcagcgcatcgccttctatcgccttcttgacgagttcttctgagcgggactctggggttcgaaatgaccgaccaagcgacgcccaacctgccatcacgagatttcgattccaccgccgccttctatgaaaggttgggcttcggaatcgttttccgggacgccggctggatgatcctccagcgcggggatctcatgctggagttcttcgcccaccccaacttgtttattgcagcttataatggttacaaataaagcaatagcatcacaaatttcacaaataaagcatttttttcactgcattctagttgtggtttgtccaaactcatcaatgtatcttatcatgtctgtataccgtcgacctctagctagagcttggcgtaatcatggtcatagctgtttcctgtgtgaaattgttatccgctcacaattccacacaacatacgagccggaagcataaagtgtaaagcctggggtgcctaatgagtgagctaactcacattaattgcgttgcgctcactgcccgctttccagtcgggaaacctgtcgtgccagctgcattaatgaatcggccaacgcgcggggagaggcggtttgcgtattgggcgctcttccgcttcctcgctcactgactcgctgcgctcggtcgttcggctgcggcgagcggtatcagctcactcaaaggcggtaatacggttatccacagaatcaggggataacgcaggaaagaacatgtgagcaaaaggccagcaaaaggccaggaaccgtaaaaaggccgcgttgctggcgtttttccataggctccgcccccctgacgagcatcacaaaaatcgacgctcaagtcagaggtggcgaaacccgacaggactataaagataccaggcgtttccccctggaagctccctcgtgcgctctcctgttccgaccctgccgcttaccggatacctgtccgcctttctcccttcgggaagcgtggcgctttctcatagctcacgctgtaggtatctcagttcggtgtaggtcgttcgctccaagctgggctgtgtgcacgaaccccccgttcagcccgaccgctgcgccttatccggtaactatcgtcttgagtccaacccggtaagacacgacttatcgccactggcagcagccactggtaacaggattagcagagcgaggtatgtaggcggtgctacagagttcttgaagtggtggcctaactacggctacactagaagaacagtatttggtatctgcgctctgctgaagccagttaccttcggaaaaagagttggtagctcttgatccggcaaacaaaccaccgctggtagcggtttttttgtttgcaagcagcagattacgcgcagaaaaaaaggatctcaagaagatcctttgatcttttctacggggtctgacgctcagtggaacgaaaactcacgttaagggattttggtcatgagattatcaaaaaggatcttcacctagatccttttaaattaaaaatgaagttttaaatcaatctaaagtatatatgagtaaacttggtctgacagttaccaatgcttaatcagtgaggcacctatctcagcgatctgtctatttcgttcatccatagttgcctgactccccgtcgtgtagataactacgatacgggagggcttaccatctggccccagtgctgcaatgataccgcgagacccacgctcaccggctccagatttatcagcaataaaccagccagccggaagggccgagcgcagaagtggtcctgcaactttatccgcctccatccagtctattaattgttgccgggaagctagagtaagtagttcgccagttaatagtttgcgcaacgttgttgccattgctacaggcatcgtggtgtcacgctcgtcgtttggtatggcttcattcagctccggttcccaacgatcaaggcgagttacatgatcccccatgttgtgcaaaaaagcggttagctccttcggtcctccgatcgttgtcagaagtaagttggccgcagtgttatcactcatggttatggcagcactgcataattctcttactgtcatgccatccgtaagatgcttttctgtgactggtgagtactcaaccaagtcattctgagaatagtgtatgcggcgaccgagttgctcttgcccggcgtcaatacgggataataccgcgccacatagcagaactttaaaagtgctcatcattggaaaacgttcttcggggcgaaaactctcaaggatcttaccgctgttgagatccagttcgatgtaacccactcgtgcacccaactgatcttcagcatcttttactttcaccagcgtttctgggtgagcaaaaacaggaaggcaaaatgccgcaaaaaagggaataagggcgacacggaaatgttgaatactcatactcttcctttttcaatattattgaagcatttatcagggttattgtctcatgagcggatacatatttgaatgtatttagaaaaataaacaaataggggttccgcgcacatttccccgaaaagtgccacctgacgtc

SEQ ID NO: 14 - DNA, 5093 bp, Artificial Sequence
  pCMV.DsRedexp.hU6.sgRNA.BsmBI-Stuffer.TS(2x).inc.pA
  promoter 1..589: /note="human cytomegalovirus (CMV) immediate early promoter"
  CDS 628..1305: /note="human-codon optimized Discosoma sp Red Fluorescent Protien (DsRed-Express)" /transl_table=1
  promoter 1313..1556: /note="human U6 promoter"
  misc_feature 1560..1668: /note="BsmBI stuffer"
  misc_feature 1669..1850: /note="sgRNA.TS.adj scaffold"
  misc_feature 1755..1775: /note="TS hairpin"
  misc_feature 1794..1814: /note="TS hairpin"
  terminator 1851..1855: /note="termination signal"
  polyA_signal 1912..1917: /note="SV40 early mRNA polyadenylation signal"
  polyA_signal 1941..1946: /note="SV40 early mRNA polyadenylation signal"
  misc_feature 2009..2464: /note="F1 single-strand DNA origin in antisense orientation"
  promoter 2526..2554: /note="bacterial beta-lactamase promoter for expression of Kanamycin resistance gene"
  promoter 2622..2867: /note="SV40 early promoter, overlaps with SV40 ori"
  misc_feature 2805..2940: /note="SV40 origin of replication"
  gene 2989..3783: /note="Kanamycin/neomycin resistance gene"
  polyA_signal 4015..4061: /note="herpes simplex virus thymidine kinase (TK) polyadenylation signal"
  misc_feature 4368..5011: /note="pUC plasmid replication origin"
tagttattaatagtaatcaattacggggtcattagttcatagcccatatatggagttccgcgttacataacttacggtaaatggcccgcctggctgaccgcccaacgacccccgcccattgacgtcaataatgacgtatgttcccatagtaacgccaatagggactttccattgacgtcaatgggtggagtatttacggtaaactgcccacttggcagtacatcaagtgtatcatatgccaagtacgccccctattgacgtcaatgacggtaaatggcccgcctggcattatgcccagtacatgaccttatgggactttcctacttggcagtacatctacgtattagtcatcgctattaccatggtgatgcggttttggcagtacatcaatgggcgtggatagcggtttgactcacggggatttccaagtctccaccccattgacgtcaatgggagtttgttttggcaccaaaatcaacgggactttccaaaatgtcgtaacaactccgccccattgacgcaaatgggcggtaggcgtgtacggtgggaggtctatataagcagagctggtttagtgaaccgtcagatccgctagcgctaccggactcagatccaccggtcgccaccatggcctcctccgaggacgtcatcaaggagttcatgcgcttcaaggtgcgcatggagggctccgtgaacggccacgagttcgagatcgagggcgagggcgagggccgcccctacgagggcacccagaccgccaagctgaaggtgaccaagggcggccccctgcccttcgcctgggacatcctgtccccccagttccagtacggctccaaggtgtacgtgaagcaccccgccgacatccccgactacaagaagctgtccttccccgagggcttcaagtgggagcgcgtgatgaacttcgaggacggcggcgtggtgaccgtgacccaggactcctccctgcaggacggctccttcatctacaaggtgaagttcatcggcgtgaacttcccctccgacggccccgtaatgcagaagaagactatgggctgggaggcctccaccgagcgcctgtacccccgcgacggcgtgctgaagggcgagatccacaaggccctgaagctgaaggacggcggccactacctggtggagttcaagtccatctacatggccaagaagcccgtgcagctgcccggctactactacgtggactccaagctggacatcacctcccacaacgaggactacaccatcgtggagcagtacgagcgcgccgagggccgccaccacctgttcctgtagcggccgcgagagggcctatttcccatgattccttcatatttgcatatacgatacaaggctgttagagagataattagaattaatttgactgtaaacacaaagatattagtacaaaatacgtgacgtagaaagtaataatttcttgggtagtttgcagttttaaaattatgttttaaaatggactatcatatgcttaccgtaacttgaaagtatttcgatttcttggctttatatatcttgtggaaaggacgaaacaccggagacggttgtaaatgagcacacaaaatacacatgctaaaatattatattctatgatttttaaatcttttttagcttcttgctcttttttgtacgtctctgttttagagctagaaatagcaagttaaaataaggctagtccgttatcaacttgaaaaagtggcaccgagtcggtgcctaattgcctagaaaacatgaggatcacccatgtctgcaggtcgactctagaaaacatgaggatcacccatgtctgcagtattcccgggttcattagatcctaaggtacttttttgaattctaccggaattgttgttgttaacttgtttattgcagcttataatggttacaaataaagcaatagcatcacaaatttcacaaataaagcatttttttcactgcattctagttgtggtttgtccaaactcatcaatgtatcttaaggcgtaaattgtaagcgttaatattttgttaaaattcgcgttaaatttttgttaaatcagctcattttttaaccaataggccgaaatcggcaaaatcccttataaatcaaaagaatagaccgagatagggttgagtgttgttccagtttggaacaagagtccactattaaagaacgtggactccaacgtcaaagggcgaaaaaccgtctatcagggcgatggcccactacgtgaaccatcaccctaatcaagttttttggggtcgaggtgccgtaaagcactaaatcggaaccctaaagggagcccccgatttagagcttgacggggaaagccggcgaacgtggcgagaaaggaagggaagaaagcgaaaggagcgggcgctagggcgctggcaagtgtagcggtcacgctgcgcgtaaccaccacacccgccgcgcttaatgcgccgctacagggcgcgtcaggtggcacttttcggggaaatgtgcgcggaacccctatttgtttatttttctaaatacattcaaatatgtatccgctcatgagacaataaccctgataaatgcttcaataatattgaaaaaggaagagtcctgaggcggaaagaaccagctgtggaatgtgtgtcagttagggtgtggaaagtccccaggctccccagcaggcagaagtatgcaaagcatgcatctcaattagtcagcaaccaggtgtggaaagtccccaggctccccagcaggcagaagtatgcaaagcatgcatctcaattagtcagcaaccatagtcccgcccctaactccgcccatcccgcccctaactccgcccagttccgcccattctccgccccatggctgactaattttttttatttatgcagaggccgaggccgcctcggcctctgagctattccagaagtagtgaggaggcttttttggaggcctaggcttttgcaaagatcgatcaagagacaggatgaggatcgtttcgcatgattgaacaagatggattgcacgcaggttctccggccgcttgggtggagaggctattcggctatgactgggcacaacagacaatcggctgctctgatgccgccgtgttccggctgtcagcgcaggggcgcccggttctttttgtcaagaccgacctgtccggtgccctgaatgaactgcaagacgaggcagcgcggctatcgtggctggccacgacgggcgttccttgcgcagctgtgctcgacgttgtcactgaagcgggaagggactggctgctattgggcgaagtgccggggcaggatctcctgtcatctcaccttgctcctgccgagaaagtatccatcatggctgatgcaatgcggcggctgcatacgcttgatccggctacctgcccattcgaccaccaagcgaaacatcgcatcgagcgagcacgtactcggatggaagccggtcttgtcgatcaggatgatctggacgaagagcatcaggggctcgcgccagccgaactgttcgccaggctcaaggcgagcatgcccgacggcgaggatctcgtcgtgacccatggcgatgcctgcttgccgaatatcatggtggaaaatggccgcttttctggattcatcgactgtggccggctgggtgtggcggaccgctatcaggacatagcgttggctacccgtgatattgctgaagagcttggcggcgaatgggctgaccgcttcctcgtgctttacggtatcgccgctcccgattcgcagcgcatcgccttctatcgccttcttgacgagttcttctgagcgggactctggggttcgaaatgaccgaccaagcgacgcccaacctgccatcacgagatttcgattccaccgccgccttctatgaaaggttgggcttcggaatcgttttccgggacgccggctggatgatcctccagcgcggggatctcatgctggagttcttcgcccaccctagggggaggctaactgaaacacggaaggagacaataccggaaggaacccgcgctatgacggcaataaaaagacagaataaaacgcacggtgttgggtcgtttgttcataaacgcggggttcggtcccagggctggcactctgtcgataccccaccgagaccccattggggccaatacgcccgcgtttcttccttttccccaccccaccccccaagttcgggtgaaggcccagggctcgcagccaacgtcggggcggcaggccctgccatagcctcaggttactcatatatactttagattgatttaaaacttcatttttaatttaaaaggatctaggtgaagatcctttttgataatctcatgaccaaaatcccttaacgtgagttttcgttccactgagcgtcagaccccgtagaaaagatcaaaggatcttcttgagatcctttttttctgcgcgtaatctgctgcttgcaaacaaaaaaaccaccgctaccagcggtggtttgtttgccggatcaagagctaccaactctttttccgaaggtaactggcttcagcagagcgcagataccaaatactgtccttctagtgtagccgtagttaggccaccacttcaagaactctgtagcaccgcctacatacctcgctctgctaatcctgttaccagtggctgctgccagtggcgataagtcgtgtcttaccgggttggactcaagacgatagttaccggataaggcgcagcggtcgggctgaacggggggttcgtgcacacagcccagcttggagcgaacgacctacaccgaactgagatacctacagcgtgagctatgagaaagcgccacgcttcccgaagggagaaaggcggacaggtatccggtaagcggcagggtcggaacaggagagcgcacgagggagcttccagggggaaacgcctggtatctttatagtcctgtcgggtttcgccacctctgacttgagcgtcgatttttgtgatgctcgtcaggggggcggagcctatggaaaaacgccagcaacgcggcctttttacggttcctggccttttgctggccttttgctcacatgttctttcctgcgttatcccctgattctgtggataaccgtattaccgccatgcat

SEQ ID NO: 15 - protein, 151 aa, Artificial Sequence
  [CDS]:1462..1914 from SEQ ID NO 1
MEAVIKVISSACKTYCGKISPSKKEIGAMLSLLQKEGLLMSPSDLYSPGSWDPITAALSQRAMVLGKSGELKTWGLVLGALKAAREEQVTSEQAKFWLGLGGGRVSPPGPECIEKPATERRIDKGEEVGETTVQRDAKMAPEEAATPKTVG

SEQ ID NO: 16 - protein, 17 aa, Artificial Sequence
  [CDS]:1936..1986 from SEQ ID NO 1
TAVGCNCATATASAPPP

SEQ ID NO: 17 - protein, 55 aa, Artificial Sequence
  [CDS]:2008..2172 from SEQ ID NO 1
YPSLAGVGEQQGQGDNTSRGAEQPREEPGHAGQAPGPALTDWARVREELASTGPP

SEQ ID NO: 18 - protein, 242 aa, Artificial Sequence
  [CDS]:2194..2919 from SEQ ID NO 1
IKTEGPAWTPLEPKLITRLADTVRTKGLRSPITMAEVEALMSSPLLPHDVTNLMRVILGPAPYALWMDAWGVQLQTVIAAATRDPRHPANGQGRGERTNLDRLKGLADGMVGNPQGQAALLRPGELVAITASALQAFREVARLAEPAGPWADITQGPSESFVDFANRLIKAVEGSDLPPSARAPVIIDCFRQKSQPDIQQLIRAAPSTLTTPGEIIKYVLDRQKIAPLTDQGIAAAMSSAIQ

SEQ ID NO: 19 - protein, 82 aa, Artificial Sequence
  [CDS]:2941..3186 from SEQ ID NO 1
NRERDGQTGSGGRARGLCYTCGSPGHYQAQCPKKRKSGNSRERCQLCDGMGHNAKQCRKRDGNQGQRPGRGLSSGPWPGPEQ

SEQ ID NO: 20 - protein, 7 aa, Artificial Sequence
  [CDS]:1915..1935 from SEQ ID NO 1
TSCYHCG

SEQ ID NO: 21 - protein, 7 aa, Artificial Sequence
  [CDS]:1987..2007 from SEQ ID NO 1
PYVGSGL

SEQ ID NO: 22 - protein, 7 aa, Artificial Sequence
  [CDS]:2173..2193 from SEQ ID NO 1
VVAMPVV

SEQ ID NO: 23 - protein, 7 aa, Artificial Sequence
  [CDS]:2920..2940 from SEQ ID NO 1
PLVMAVV

SEQ ID NO: 24 - protein, 7 aa, Artificial Sequence
  [CDS]:3187..3207 from SEQ ID NO 1
PAVSLAM

SEQ ID NO: 25 - protein, 5 aa, Artificial Sequence
  [CDS]:3208..3222 from SEQ ID NO 1
TGGGG

SEQ ID NO: 26 - protein, 258 aa, Artificial Sequence
  [CDS]:3223..3999 from SEQ ID NO 1
MASNFTQFVLVDNGGTGDVTVAPSNFANGVAEWISSNSRSQAYKVTCSVRQSSAQNRKYTIKVEVPKVATQTVGGVELPVAAWRSYLNMELTIPIFATNSDCELIVKAMQGLLKDGNPIPSAIAANSGIYANFTQFVLVDNGGTGDVTVAPSNFANGVAEWISSNSRSQAYKVTCSVRQSSAQNRKYTIKVEVPKVATQTVGGVELPVAAWRSYLNMELTIPIFATNSDCELIVKAMQGLLKDGNPIPSAIAANSGIY

SEQ ID NO: 27 - protein, 135 aa, Artificial Sequence
  [CDS]:3208..3612 from SEQ ID NO 1
TGGGGMASNFTQFVLVDNGGTGDVTVAPSNFANGVAEWISSNSRSQAYKVTCSVRQSSAQNRKYTIKVEVPKVATQTVGGVELPVAAWRSYLNMELTIPIFATNSDCELIVKAMQGLLKDGNPIPSAIAANSGIY

SEQ ID NO: 28 - protein, 127 aa, Artificial Sequence
  [CDS]:3616..3999 from SEQ ID NO 1
NFTQFVLVDNGGTGDVTVAPSNFANGVAEWISSNSRSQAYKVTCSVRQSSAQNRKYTIKVEVPKVATQTVGGVELPVAAWRSYLNMELTIPIFATNSDCELIVKAMQGLLKDGNPIPSAIAANSGIY

SEQ ID NO: 29 - protein, 264 aa, Artificial Sequence [sequence omitted]

SEQ ID NO: 30 - protein, 432 aa, Artificial Sequence
  [CDS]:612..1910 from SEQ ID NO 2
MAPKKKRKVMSQFDILCKTPPKVLVRQFVERFERPSGEKIASCAAELTYLCWMITHNGTAIKRATFMSYNTIISNSLSFDIVNKSLQFKYKTQKATILEASLKKLIPAWEFTIIPYNGQKHQSDITDIVSSLQLQFESSEEADKGNSHSKKMLKALLSEGESIWEITEKILNSFEYTSRFTKTKTLYQFLFLATFINCGRFSDIKNVDPKSFKLVQNKYLGVIIQCLVTETKTSVSRHIYFFSARGRIDPLVYLDEFLRNSEPVLKRVNRTGNSSSNKQEYQLLKDNLVRSYNKALKKNAPYPIFAIKNGPKSHIGRHLMTSFLSMKGLTELTNVVGNWSDKRASAVARTTYTHQITAIPDHYFALVSRYYAYDPISKEMIALKDETNPIEEWQHIEQLKGSAEGSIRYPAWNGIISQEVLDYLSSYINRRI

SEQ ID NO: 31 - protein, 225 aa, Artificial Sequence
  [CDS]:628..1305 from SEQ ID NO 3
MASSEDVIKEFMRFKVRMEGSVNGHEFEIEGEGEGRPYEGTQTAKLKVTKGGPLPFAWDILSPQFQYGSKVYVKHPADIPDYKKLSFPEGFKWERVMNFEDGGVVTVTQDSSLQDGSFIYKVKFIGVNFPSDGPVMQKKTMGWEASTERLYPRDGVLKGEIHKALKLKDGGHYLVEFKSIYMAKKPVQLPGYYYVDSKLDITSHNEDYTIVEQYERAEGRHHLFL

SEQ ID NO: 32 - protein, 511 aa, Artificial Sequence
  [CDS]:1241..2776 from SEQ ID NO 4
MKCLLYLAFLFIGVNCKFTIVFPHNQKGNWKNVPSNYHYCPSSSDLNWHNDLIGTALQVKMPKSHKAIQADGWMCHASKWVTTCDFRWYGPKYITHSIRSFTPSVEQCKESIEQTKQGTWLNPGFPPQSCGYATVTDAEAVIVQVTPHHVLVDEYTGEWVDSQFINGKCSNYICPTVHNSTTWHSDYKVKGLCDSNLISMDITFFSEDGELSSLGKEGTGFRSNYFAYETGGKACKMQYCKHWGVRLPSGVWFEMADKDLFAAARFPECPEGSSISAPSQTSVDVSLIQDVERILDYSLCQETWSKIRAGLPISPVDLSYLAPKNPGTGPAFTIINGTLKYFETRYIRVDIAAPILSRMVGMISGTTTERELWDDWAPYEDVEIGPNGVLRTSSGYKFPLYMIGHGMLDSDLHLSSKAQVFEHPHIQDAASQLPDDESLFFGDTGLSKNPIELVEGWFSSWKSSIASFFFIIGLIIGLFLVLRVGIHLCIKLKHTKKRQIYTDIEMNRLGK

SEQ ID NO: 33 - protein, 1409 aa, Artificial Sequence
  [CDS]:612..4838 from SEQ ID NO 5
MDYKDDDDKMAPKKKRKVGIHGVPAADKKYSIGLDIGTNSVGWAVITDEYKVPSKKFKVLGNTDRHSIKKNLIGALLFDSGETAEATRLKRTARRRYTRRKNRICYLQEIFSNEMAKVDDSFFHRLEESFLVEEDKKHERHPIFGNIVDEVAYHEKYPTIYHLRKKLVDSTDKADLRLIYLALAHMIKFRGHFLIEGDLNPDNSDVDKLFIQLVQTYNQLFEENPINASGVDAKAILSARLSKSRRLENLIAQLPGEKKNGLFGNLIALSLGLTPNFKSNFDLAEDAKLQLSKDTYDDDLDNLLAQIGDQYADLFLAAKNLSDAILLSDILRVNTEITKAPLSASMIKRYDEHHQDLTLLKALVRQQLPEKYKEIFFDQSKNGYAGYIDGGASQEEFYKFIKPILEKMDGTEELLVKLNREDLLRKQRTFDNGSIPHQIHLGELHAILRRQEDFYPFLKDNREKIEKILTFRIPYYVGPLARGNSRFAWMTRKSEETITPWNFEEVVDKGASAQSFIERMTNFDKNLPNEKVLPKHSLLYEYFTVYNELTKVKYVTEGMRKPAFLSGEQKKAIVDLLFKTNRKVTVKQLKEDYFKKIECFDSVEISGVEDRFNASLGTYHDLLKIIKDKDFLDNEENEDILEDIVLTLTLFEDREMIEERLKTYAHLFDDKVMKQLKRRRYTGWGRLSRKLINGIRDKQSGKTILDFLKSDGFANRNFMQLIHDDSLTFKEDIQKAQVSGQGDSLHEHIANLAGSPAIKKGILQTVKVVDELVKVMGRHKPENIVIEMARENQTTQKGQKNSRERMKRIEEGIKELGSQILKEHPVENTQLQNEKLYLYYLQNGRDMYVDQELDINRLSDYDVDHIVPQSFLKDDSIDNKVLTRSDKNRGKSDNVPSEEVVKKMKNYWRQLLNAKLITQRKFDNLTKAERGGLSELDKAGFIKRQLVETRQITKHVAQILDSRMNTKYDENDKLIREVKVITLKSKLVSDFRKDFQFYKVREINNYHHAHDAYLNAVVGTALIKKYPKLESEFVYGDYKVYDVRKMIAKSEQEIGKATAKYFFYSNIMNFFKTEITLANGEIRKRPLIETNGETGEIVWDKGRDFATVRKVLSMPQVNIVKKTEVQTGGFSKESILPKRNSDKLIARKKDWDPKKYGGFDSPTVAYSVLVVAKVEKGKSKKLKSVKELLGITIMERSSFEKNPIDFLEAKGYKEVKKDLIIKLPKYSLFELENGRKRMLASAGELQKGNELALPSKYVNFLYLASHYEKLKGSPEDNEQKQLFVEQHKHYLDEIIEQISEFSKRVILADANLDKVLSAYNKHRDKPIREQAENIIHLFTLTNLGAPAAFKYFDTTIDRKRYTSTKEVLDATLIHQSITGLYETRIDLSQLGGDKRPAATKKAGQAKKKK

SEQ ID NO: 34 - protein, 8 aa, Artificial Sequence
  [CDS]:615..638 from SEQ ID NO 5
DYKDDDDK

SEQ ID NO: 35 - protein, 7 aa, Artificial Sequence
  [CDS]:645..665 from SEQ ID NO 5
PKKKRKV

SEQ ID NO: 36 - protein, 16 aa, Artificial Sequence
  [CDS]:4791..4838 from SEQ ID NO 5
KRPAATKKAGQAKKKK

SEQ ID NO: 37 - protein, 22 aa, Artificial Sequence
  [CDS]:4845..4910 from SEQ ID NO 5
GSGATNFSLLKQAGDVEENPGP

SEQ ID NO: 38 - protein, 264 aa, Artificial Sequence
  [CDS]:7988..8782 from SEQ ID NO 5
MIEQDGLHAGSPAAWVERLFGYDWAQQTIGCSDAAVFRLSAQGRPVLFVKTDLSGALNELQDEAARLSWLATTGVPCAAVLDVVTEAGRDWLLLGEVPGQDLLSSHLAPAEKVSIMADAMRRLHTLDPATCPFDHQAKHRIERARTRMEAGLVDQDDLDEEHQGLAPAELFARLKASMPDGEDLVVTHGDACLPNIMVENGRFSGFIDCGRLGVADRYQDIALATRDIAEELGGEWADRFLVLYGIAAPDSQRIAFYRLLDEFF

SEQ ID NO: 39 - protein, 239 aa, Artificial Sequence
  [CDS]:4911..5630 from SEQ ID NO 5
MVSKGEELFTGVVPILVELDGDVNGHKFSVSGEGEGDATYGKLTLKFICTTGKLPVPWPTLVTTLTYGVQCFSRYPDHMKQHDFFKSAMPEGYVQERTIFFKDDGNYKTRAEVKFEGDTLVNRIELKGIDFKEDGNILGHKLEYNYNSHNVYIMADKQKNGIKVNFKIRHNIEDGSVQLADHYQQNTPIGDGPVLLPDNHYLSTQSALSKDPNEKRDHMVLLEFVTAAGITLGMDELYK

SEQ ID NO: 40 - protein, 550 aa, Artificial Sequence
  [CDS]:624..2276 from SEQ ID NO 6
MEDAKNIKKGPAPFYPLEDGTAGEQLHKAMKRYALVPGTIAFTDAHIEVDITYAEYFEMSVRLAEAMKRYGLNTNHRIVVCSENSLQFFMPVLGALFIGVAVAPANDIYNERELLNSMGISQPTVVFVSKKGLQKILNVQKKLPIIQKIIIMDSKTDYQGFQSMYTFVTSHLPPGFNEYDFVPESFDRDKTIALIMNSSGSTGLPKGVALPHRTACVRFSHARDPIFGNQIIPDTAILSVVPFHHGFGMFTTLGYLICGFRVVLMYRFEEELFLRSLQDYKIQSALLVPTLFSFFAKSTLIDKYDLSNLHEIASGGAPLSKEVGEAVAKRFHLPGIRQGYGLTETTSAILITPEGDDKPGAVGKVVPFFEAKVVDLDTGKTLGVNQRGELCVRGPMIMSGYVNNPEATNALIDKDGWLHSGDIAYWDEDEHFFIVDRLKSLIKYKGYQVAPAELESILLQHPNIFDAGVAGLPDDDAGELPAAVVVLEHGKTMTEKEIVDYVASQVTTAKKLRGGVVFVDEVPKGLTGKLDARKIREILIKAKKGGKIAV

SEQ ID NO: 41 - protein, 151 aa, Artificial Sequence; identical to SEQ ID NO: 15
  [CDS]:1462..1914 from SEQ ID NO 12

SEQ ID NO: 42 - protein, 17 aa, Artificial Sequence
  [CDS]:1936..1986 from SEQ ID NO 12
TAVGCNCATATASAPPP

SEQ ID NO: 43 - protein, 55 aa, Artificial Sequence; identical to SEQ ID NO: 17
  [CDS]:2008..2172 from SEQ ID NO 12

SEQ ID NO: 44 - protein, 242 aa, Artificial Sequence; identical to SEQ ID NO: 18
  [CDS]:2194..2919 from SEQ ID NO 12

SEQ ID NO: 45 - protein, 82 aa, Artificial Sequence; identical to SEQ ID NO: 19
  [CDS]:2941..3186 from SEQ ID NO 12

SEQ ID NO: 46 - protein, 122 aa, Artificial Sequence
  [CDS]:3208..3573 from SEQ ID NO 12
TMEHKDRPLVRVILTNTGSHPVKQRSVYITALLDSGADITIISEEDWPTDWPVVDTANPQIHGIGGGIPMRKSRDMIEVGVINRDGSLERPLLLFPAVAMVRGSILGRDCLQGLGLRLTNLR

SEQ ID NO: 47 - protein, 7 aa, Artificial Sequence
  [CDS]:1915..1935 from SEQ ID NO 12
TSCYHCG

SEQ ID NO: 48 - protein, 7 aa, Artificial Sequence
  [CDS]:1987..2007 from SEQ ID NO 12
PYVGSGL

SEQ ID NO: 49 - protein, 7 aa, Artificial Sequence
  [CDS]:2173..2193 from SEQ ID NO 12
VVAMPVV

SEQ ID NO: 50 - protein, 7 aa, Artificial Sequence
  [CDS]:2920..2940 from SEQ ID NO 12
PLVMAVV

SEQ ID NO: 51 - protein, 7 aa, Artificial Sequence
  [CDS]:3187..3207 from SEQ ID NO 12
PAVSLAM

SEQ ID NO: 52 - protein, 7 aa, Artificial Sequence
  [CDS]:3574..3594 from SEQ ID NO 12
ATVLTVA

SEQ ID NO: 53 - protein, 6 aa, Artificial Sequence
  [CDS]:3595..3612 from SEQ ID NO 12
LTGGGG

SEQ ID NO: 54 - protein, 258 aa, Artificial Sequence; identical to SEQ ID NO: 26
  [CDS]:3613..4389 from SEQ ID NO 12

SEQ ID NO: 55 - protein, 130 aa, Artificial Sequence
  [CDS]:3613..4002 from SEQ ID NO 12
MASNFTQFVLVDNGGTGDVTVAPSNFANGVAEWISSNSRSQAYKVTCSVRQSSAQNRKYTIKVEVPKVATQTVGGVELPVAAWRSYLNMELTIPIFATNSDCELIVKAMQGLLKDGNPIPSAIAANSGIY

SEQ ID NO: 56 - protein, 127 aa, Artificial Sequence; identical to SEQ ID NO: 28
  [CDS]:4006..4389 from SEQ ID NO 12

SEQ ID NO: 57 - protein, 481 aa, Artificial Sequence
  [CDS]:1475..2917 from SEQ ID NO 13
MGQTVTTPLSLTLGHWKDVERIAHNQSVDVKKRRWVTFCSAEWPTFNVGWPRDGTFNRDLITQVKIKVFSPGPHGHPDQVPYIVTWEALAFDPPPWVKPFVHPKPPPPLPPSAPSLPLEPPRSTPPRSSLYPALTPSLGAKPKPQVLSDSGGPLIDLLTEDPPPYRDPRPPPSDRDGNGGEATPAGEAPDPSPMASRLRGRREPPVADSTTSQAFPLRAGGNGQLQYWPFSSSDLYNWKNNNPSFSEDPGKLTALIESVLITHQPTWDDCQQLLGTLLTGEEKQRVLLEARKAVRGDDGRPTQLPNEVDAAFPLERPDWDYTTQAGRNHLVHYRQLLLAGLQNAGRSPTNLAKVKGITQGPNESPSAFLERLKEAYRRYTPYDPEDPGQETNVSMSFIWQSAPDIGRKLERLEDLKNKTLGDLVREAEKIFNKRETPEEREERIRRETEEKEERRRTEDEQKEKERDRRRHREMSKLLATV

SEQ ID NO: 58 - protein, 127 aa, Artificial Sequence
  [CDS]:1475..1855 from SEQ ID NO 13
MGQTVTTPLSLTLGHWKDVERIAHNQSVDVKKRRWVTFCSAEWPTFNVGWPRDGTFNRDLITQVKIKVFSPGPHGHPDQVPYIVTWEALAFDPPPWVKPFVHPKPPPPLPPSAPSLPLEPPRSTPPR

SEQ ID NO: 59 - protein, 77 aa, Artificial Sequence
  [CDS]:1877..2107 from SEQ ID NO 13
TPSLGAKPKPQVLSDSGGPLIDLLTEDPPPYRDPRPPPSDRDGNGGEATPAGEAPDPSPMASRLRGRREPPVADSTT

SEQ ID NO: 60 - protein, 256 aa, Artificial Sequence
  [CDS]:2129..2896 from SEQ ID NO 13
AGGNGQLQYWPFSSSDLYNWKNNNPSFSEDPGKLTALIESVLITHQPTWDDCQQLLGTLLTGEEKQRVLLEARKAVRGDDGRPTQLPNEVDAAFPLERPDWDYTTQAGRNHLVHYRQLLLAGLQNAGRSPTNLAKVKGITQGPNESPSAFLERLKEAYRRYTPYDPEDPGQETNVSMSFIWQSAPDIGRKLERLEDLKNKTLGDLVREAEKIFNKRETPEEREERIRRETEEKEERRRTEDEQKEKERDRRRHREM

SEQ ID NO: 61 - protein, 258 aa, Artificial Sequence; identical to SEQ ID NO: 26
  [CDS]:2936..3712 from SEQ ID NO 13

SEQ ID NO: 62 - protein, 225 aa, Artificial Sequence; identical to SEQ ID NO: 31
  [CDS]:628..1305 from SEQ ID NO 14